European Patent Application EP 4 745 236 A1, published May 20, 2026. Title: 工程化的哺乳动物基因写入系统. Applicant: 北京干细胞与再生医学研究院. The sequence listing filed with the application follows.

SEQUENCE LISTING (89 sequences)

SEQ ID NO: 1 - protein, 1390 aa, synthetic construct
MASCPKPGPPVSAGAMSLESGLTTHSVLAIERGPNSLANSGSDFGGGGLGLPLRLLRVSVGTQTSRSDWVDLVSWSHPGPTSKSQQVDLVSLFPKHRVDLLSKNDQVDLVAQFLPSKFPPNLAENDLALLVNLEFYRSDLHVYECVHFAAHWEGLSGLPEVYEQLAPQPCVGETLHSSLPRDSELFVPEEGSSEKESEDAPKTSPPTPGKHGLEQTGEEKVMVTVPDKNPPCPCCGTRVNSVLNLIEHLKVSHGKRGVCFRCAKCGKENSNYHSVVCHFPKCRGPETEKAPAGEWICEVCNRDFTTKIGLGQHKRLAHPAVRNQERIVASQPKETSNRGAHKRCWTKEEEELLIRLEAQFEGNKNINKLIAEHITTKTAKQISDKRRLLSRKPAEEPREEPGTCHHTRRAAASLRTEPEMSHHAQAEDRDNGPGRRPLPGRAAAGGRTMDEIRRHPDKGNGQQRPTKQKSEEQLQAYYKKTLEERLSAGALNTFPRAFKQVMEGRDIKLVINQTAQDCFGCLESISQIRTATRDKKDTVTREKHPKKPFQKWMKDRAIKKGNYLRFQRLFYLDRGKLAKIILDDIECLSCDIPLSEIYSVFKTRWETTGSFKSLGDFKTYGKADNTAFRELITAKEIEKNVQEMSKGSAPGPDGITLGDVVKMDPEFSRTMEIFNLWLTTGKIPDMVRGCRTVLIPKSSKPDRLKDINNWRPITIGSILLRLFSRIVTARLSKACPLNPRQRGFIRAAGCSENLKLLQTIIWSAKREHRPLGVVFVDIAKAFDTVSHQHIIHALQQREVDPHIVGLVSNMYENISTYITTKRNTHTDKIQIRVGVKQGDPMSPLLFNLAMDPLLCKLEESGKGYHRGQSSITAMAFADDLVLLSDSWENMNTNISILETFCNLTGLKTQGQKCHGFYIKPTKDSYTINDCAAWTINGTPLNMIDPGESEKYLGLQFDPWIGIARSGLSTKLDFWLQRIDQAPLKPLQKTDILKTYTIPRLIYIADHSEVKTALLETLDQKIRTAVKEWLHLPPCTCDAILYSSTRDGGLGITKLAGLIPSVQARRLHRIAQSSDDTMKCFMEKEKMEQLHKKLWIQAGGDRENIPSIWEAPPSSEPPNNVSTNSEWEAPTQKDKFPKPCNWRKNEFKKWTKLASQGRGIVNFERDKISNHWIQYYRRIPHRKLLTALQLRANVYPTREFLARGRQDQYIKACRHCDADIESCAHIIGNCPVTQDARIKRHNYICELLLEEAKKKDWVVFKEPHIRDSNKELYKPDLIFVKDARALVVDVTVRYEAAKSSLEEAAAEKVRKYKHLETEVRHLTNAKDVTFVGFPLGARGKWHQDNFKLLTELGLSKSRQVKMAETFSTVALFSSVDIVHMFASRARKSMVM

SEQ ID NO: 2 - protein, 1390 aa, synthetic construct
MASCPKPGPPVSAGAMSLESGLTTHSVLAIERGPNSLANSGSDFGGGGLGLPLRLLRVSVGTQTSRSDWVDLVSWSHPGPTSKSQQVDLVSLFPKHRVDLLSKNDQVDLVAQFLPSKFPPNLAENDLALLVNLEFYRSDLHVYECVHFAAHWEGLSGLPEVYEQLAPQPCVGETLHSSLPRDSELFVPEEGSSEKESEDAPKTSPPTPGKHGLEQTGEEKVMVTVPDKNPPCPCCGTRVNSVLNLIEHLKVSHGKRGVCFRCAKCGKENSNYHSVVCHFPKCRGPETEKAPAGEWICEVCNRDFTTKIGLGQHKRLAHPAVRNQERIVASQPKETSNRGAHKRCWTKEEEELLIRLEAQFEGNKNINKLIAEHITTKTAKQISDKRRLLSRKPAEEPREEPGTCHHTRRAAASLRTEPEMSHHAQAEDRDNGPGRRPLPGRAAAGGRTMDEIRRHPDKGNGQQRPTKQKSEEQLQAYYKKTLEERLSAGALNTFPRAFKQVMEGRDIKLVINQTAQDCFGCLESISQIRTATRDKKDTVTREKHPKKPFQKWMKDRAIKKGNYLRFQRLFYLDRGKLAKIILDDIECLSCDIPLSEIYSVFKTRWETTGSFKSLGDFKTYGKADNTAFRELITAKEIEKNVQEMSKGSAPGPDGITLGDVVKMDPEFSRTMEIFNLWLTTGKIPDMVRGCRTVLIPKSSKPDRLKDINNWRPITIGSILLRLFSRIVTARLSKACPLNPRQRGFIRAAGCSENLKLLQTIIWSAKREHRPLGVVFVDIAKAFDTVSHQHIIHALQQREVDPHIVGLVSNMYENISTYITTKRNTHTDKIQIRVGVKQGDPMSPLLFNLAMDPLLCKLEESGKGYHRGQSSITAMAFADDLVLLSDSWENMNTNISILETFCNLTGLKTQGQKCHGFYIKPTKDSYTINDCAAWTINGTPLNMIDPGESEKYLGLQFDPWIGIARSGLSTKLDFWLQRIDQAPLKPLQKTDILKTYTIPRLIYIADHSEVKTALLETLDQKIRTAVKEWLHLPPCTCDAILYSSTRDGGLGITKLAGLIPSVQARRLHRIAQSSDDTMKCFMEKEKMEQLHKKLWIQARGDRENIPSIWEAPPSSEPPNNVSTNSEWEAPTQKDKFPKPCNWRKNEFKKWTKLASQGRGIVNFERDKISNHWIQYYRRIPHRKLLTALQLRANVYPTREFLARGRQDQYIKACRHCDADIESCAHIIGNCPVTQDARIKRHNYICELLLEEAKKKDWVVFKEPHIRDSNKELYKPDLIFVKDARALVVDVTVRYEAAKSSLEEAAAEKVRKYKHLETEVRHLTNAKDVTFVGFPLGARGKWHQDNFKLLTELGLSKSRQVKMAETFSTVALFSSVDIVHMFASRARKSMVM

SEQ ID NO: 3 - protein, 1390 aa, synthetic construct
MASCPKPGPPVSAGAMSLESGLTTHSVLAIERGPNSLANSGSDFGGGGLGLPLRLLRVSVGTQTSRSDWVDLVSWSHPGPTSKSQQVDLVSLFPKHRVDLLSKNDQVDLVAQFLPSKFPPNLAENDLALLVNLEFYRSDLHVYECVHFAAHWEGLSGLPEVYEQLAPQPCVGETLHSSLPRDSELFVPEEGSSEKESEDAPKTSPPTPGKHGLEQTGEEKVMVTVPDKNPPCPCCGTRVNSVLNLIEHLKVSHGKRGVCFRCAKCGKENSNYHSVVCHFPKCRGPETEKAPAGEWICEVCNRDFTTKIGLGQHKRLAHPAVRNQERIVASQPKETSNRGAHKRCWTKEEEELLIRLEAQFEGNKNINKLIAEHITTKTAKQISDKRRLLSRKPAEEPREEPGTCHHTRRAAASLRTEPEMSHHAQAEDRDNGPGRRPLPGRAAAGGRTMDEIRRHPDKGNGQQRPTKQKSEEQLQAYYKKTLEERLSAGALNTFPRAFKQVMEGRDIKLVINQTAQDCFGCLESISQIRTATRDKKDTVTREKHPKKPFQKWMKDRAIKKGNYLRFQRLFYLDRGKLAKIILDDIECLSCDIPLSEIYSVFKTRWETTGSFKSLGDFKTYGKADNTAFRELITAKEIEKNVQEMSKGSAPGPDGITLGDVVKMDPEFSRTMEIFNLWLTTGKIPDMVRGCRTVLIPKSSKPDRLKDINNWRPITIGSILLRLFSRIVTARLSKACPLNPRQRGFIRAAGCSENLKLLQTIIWSAKREHRPLGVVFVDIAKAFDTVSHQHIIHVLQQREVDPHIVGLVSNMYENISTYITTKRNTHTDKIQIRVGVKQGDPMSPLLFNLAMDPLLCKLEESGKGYHRGQSSITAMAFADDLVLLSDSWENMNTNISILETFCNLTGLKTQGQKCHGFYIKPTKDSYTINDCAAWTINGTPLNMIDPGESEKYLGLQFDPWIGIARSGLSTKLDFWLQRIDQAPLKPLQKTDILKTYTIPRLIYIADHSEVKTALLETLDQKIRTAVKEWLHLPPCTCDAILYSSTRDGGLGITKLAGLIPSVQARRLHRIAQSSDDTMKCFMEKEKMEQLHKKLWIQARGDRENIPSIWEAPPSSEPPNNVSTNSEWEAPTQKDKFPKPCNWRKNEFKKWTKLASQGRGIVNFERDKISNHWIQYYRRIPHRKLLTALQLRANVYPTREFLARGRQDQYIKACRHCDADIESCAHIIGNCPVTQDARIKRHNYICELLLEEAKKKDWVVFKEPHIRDSNKELYKPDLIFVKDARALVVDVTVRYEAAKSSLEEAAAEKVRKYKHLETEVRHLTNAKDVTFVGFPLGARGKWHQDNFKLLTELGLSKSRQVKMAETFSTVALFSSVDIVHMFASRARKSMVM

SEQ ID NO: 4 - protein, 1390 aa, synthetic construct
MASCPKPGPPVSAGAMSLESGLTTHSVLAIERGPNSLANSGSDFGGGGLGLPLRLLRVSVGTQTSRSDWVDLVSWSHPGPTSKSQQVDLVSLFPKHRVDLLSKNDQVDLVAQFLPSKFPPNLAENDLALLVNLEFYRSDLHVYECVHFAAHWEGLSGLPEVYEQLAPQPCVGETLHSSLPRDSELFVPEEGSSEKESEDAPKTSPPTPGKHGLEQTGEEKVMVTVPDKNPPCPCCGTRVNSVLNLIEHLKVSHGKRGVCFRCAKCGKENSNYHSVVCHFPKCRGPETEKAPAGEWICEVCNRDFTTKIGLGQHKRLAHPAVRNQERIVASQPKETSNRGAHKRCWTKEEEELLIRLEAQFEGNKNINKLIAEHITTKTAKQISDKRRLLSRKPAEEPREEPGTCHHTRRAAASLRTEPEMSHHAQAEDRDNGPGRRPLPGRAAAGGRTMDEIRRHPDKGNGQQRPTKQKSEEQLQAYYKKTLEERLSAGALNTFPRAFKQVMEGRDIKLVINQTAQDCFGCLESISQIRTATRDKKDTVTREKHPKKPFQKWMKDRAIKKGNYLRFQRLFYLDRGKLAKIILDDIECLSCDIPLSEIYSVFKTRWETTGSFKSLGDFKTYGKADNTAFRELITAKEIEKNVQEMSKGSAPGPDGITLGDVVKMDPEFSRTMEIFNLWLTTGKIPDMVRGCRTVLIPKSSKPDRLKDINNWRPITIGSILLRLFSRIVTARLSKACPLNPRQRGFIRAAGCSENLKLLQTIIWSAKREHRPLGVVFVDIAKAFDTVSHQHIIHVLQQREVDPHIVGLVSNMYENISTYITTKRNTHTDKIQIRVGVKQGDPMSPLLFNLAMDPLLCKLEESGKGYHRGQSSITAMAFADDLVLLSDSWENMNTNISILETFCNLTGLKTQGQKCHGFYIKPTKDSYTINDCAAWTINGTPLNMIDPGESEKYLGLRFDPWIGIARSGLSTKLDFWLQRIDQAPLKPLQKTDILKTYTIPRLIYIADHSEVKTALLETLDQKIRTAVKEWLHLPPCTCDAILYSSTRDGGLGITKLAGLIPSVQARRLHRIAQSSDDTMKCFMEKEKMEQLHKKLWIQARGDRENIPSIWEAPPSSEPPNNVSTNSEWEAPTQKDKFPKPCNWRKNEFKKWTKLASQGRGIVNFERDKISNHWIQYYRRIPHRKLLTALQLRANVYPTREFLARGRQDQYIKACRHCDADIESCAHIIGNCPVTQDARIKRHNYICELLLEEAKKKDWVVFKEPHIRDSNKELYKPDLIFVKDARALVVDVTVRYEAAKSSLEEAAAEKVRKYKHLETEVRHLTNAKDVTFVGFPLGARGKWHQDNFKLLTELGLSKSRQVKMAETFSTVALFSSVDIVHMFASRARKSMVM

SEQ ID NO: 5 - protein, 1390 aa, synthetic construct
MASCPKPGPPVSAGAMSLESGLTTHSVLAIERGPNSLANSGSDFGGGGLGLPLRLLRVSVGTQTSRSDWVDLVSWSHPGPTSKSQQVDLVSLFPKHRVDLLSKNDQVDLVAQFLPSKFPPNLAENDLALLVNLEFYRSDLHVYECVHFAAHWEGLSGLPEVYEQLAPQPCVGETLHSSLPRDSELFVPEEGSSEKESEDAPKTSPPTPGKHGLEQTGEEKVMVTVPDKNPPCPCCGTRVNSVLNLIEHLKVSHGKRGVCFRCAKCGKENSNYHSVVCHFPKCRGPETEKAPAGEWICEVCNRDFTTKIGLGQHKRLAHPAVRNQERIVASQPKETSNRGAHKRCWTKEEEELLIRLEAQFEGNKNINKLIAEHITTKTAKQISDKRRLLSRKPAEEPREEPGTCHHTRRAAASLRTEPEMSHHAQAEDRDNGPGRRPLPGRAAAGGRTMDEIRRHPDKGNGQQRPTKQKSEEQLQAYYKKTLEERLSAGALNTFPRAFKQVMEGRDIKLVINQTAQDCFGCLESISQIRTATRDKKDTVTREKHPKKPFQKWMKDRAIKKGNYLRFQRLFYLDRGKLAKIILDDIECLSCDIPLSEIYSVFKTRWETTGSFKSLGDFKTYGKADNTAFRELITAKEIEKNVQEMSKGSAPGPDGITLGDVVKMDPEFSRTMEIFNLWLTTGKIPDMVRGCRTVLIPKSSKPDRLKDINNWRPITIGSILLRLFSRIVTARLSKACPLNPRQRGFIRAAGCSENLKLLQTIIQSAKREHRPLGVVFVDIAKAFDTVSHQHIIHVLQQREVDPHIVGLVSNMYENISTYITTKRNTHTDKIQIRVGVKQGDPMSPLLFNLAMDPLLCKLEESGKGYHRGQSSITAMAFADDLVLLSDSWENMNTNISILETFCNLTGLKTQGQKCHGFYIKPTKDSYTINDCAAWTINGTPLNMIDPGESEKYLGLRFDPWIGIARSGLSTKLDFWLQRIDQAPLKPLQKTDILKTYTIPRLIYIADHSEVKTALLETLDQKIRTAVKEWLHLPPCTCDAILYSSTRDGGLGITKLAGLIPSVQARRLHRIAQSSDDTMKCFMEKEKMEQLHKKLWIQARGDRENIPSIWEAPPSSEPPNNVSTNSEWEAPTQKDKFPKPCNWRKNEFKKWTKLASQGRGIVNFERDKISNHWIQYYRRIPHRKLLTALQLRANVYPTREFLARGRQDQYIKACRHCDADIESCAHIIGNCPVTQDARIKRHNYICELLLEEAKKKDWVVFKEPHIRDSNKELYKPDLIFVKDARALVVDVTVRYEAAKSSLEEAAAEKVRKYKHLETEVRHLTNAKDVTFVGFPLGARGKWHQDNFKLLTELGLSKSRQVKMAETFSTVALFSSVDIVHMFASRARKSMVM

SEQ ID NO: 6 - protein, 1390 aa, synthetic construct
MASCPKPGPPVSAGAMSLESGLTTHSVLAIERGPNSLANSGSDFGGGGLGLPLRLLRVSVGTQTSRSDWVDLVSWSHPGPTSKSQQVDLVSLFPKHRVDLLSKNDQVDLVAQFLPSKFPPNLAENDLALLVNLEFYRSDLHVYECVHFAAHWEGLSGLPEVYEQLAPQPCVGETLHSSLPRDSELFVPEEGSSEKESEDAPKTSPPTPGKHGLEQTGEEKVMVTVPDKNPPCPCCGTRVNSVLNLIEHLKVSHGKRGVCFRCAKCGKENSNYHSVVCHFPKCRGPETEKAPAGEWICEVCNRDFTTKIGLGQHKRLAHPAVRNQERIVASQPKETSNRGARKRCWTKEEEELLIRLEAQFEGNKNINKLIAEHITTKTAKQISDKRRLLSRKPAEEPREEPGTCHHTRRAAASLRTEPEMSHHAQAEDRDNGPGRRPLPGRAAAGGRTMDEIRRHPDKGNGQQRPTKQKSEEQLQAYYKKTLEERLSAGALNTFPRAFKQVMEGRDIKLVINQTAQDCFGCLESISQIRTATRDKKDTVTREKHPKKPFQKWMKDRAIKKGNYLRFQRLFYLDRGKLAKIILDDIECLSCDIPLSEIYSVFKTRWETTGSFKSLGDFKTYGKADNTAFRELITAKEIEKNVQEMSKGSAPGPDGITLGDVVKMDPEFSRTMEIFNLWLTTGKIPDMVRGCRTVLIPKSSKPDRLKDINNWRPITIGSILLRLFSRIVTARLSKACPLNPRQRGFIRAAGCSENLKLLQTIIQSAKREHRPLGVVFVDIAKAFDTVSHQHIIHVLQQREVDPHIVGLVSNMYENISTYITTKRNTHTDKIQIRVGVKQGDPMSPLLFNLAMDPLLCKLEESGKGYHRGQSSITAMAFADDLVLLSDSWENMNTNISILETFCNLTGLKTQGQKCHGFYIKPTKDSYTINDCAAWTINGTPLNMIDPGESEKYLGLRFDPWIGIARSGLSTKLDFWLQRIDQAPLKPLQKTDILKTYTIPRLIYIADHSEVKTALLETLDQKIRTAVKEWLHLPPCTCDAILYSSTRDGGLGITKLAGLIPSVQARRLHRIAQSSDDTMKCFMEKEKMEQLHKKLWIQARGDRENIPSIWEAPPSSEPPNNVSTNSEWEAPTQKDKFPKPCNWRKNEFKKWTKLASQGRGIVNFERDKISNHWIQYYRRIPHRKLLTALQLRANVYPTREFLARGRQDQYIKACRHCDADIESCAHIIGNCPVTQDARIKRHNYICELLLEEAKKKDWVVFKEPHIRDSNKELYKPDLIFVKDARALVVDVTVRYEAAKSSLEEAAAEKVRKYKHLETEVRHLTNAKDVTFVGFPLGARGKWHQDNFKLLTELGLSKSRQVKMAETFSTVALFSSVDIVHMFASRARKSMVM

SEQ ID NO: 7 - protein, 1390 aa, synthetic construct
MASCPKPGPPVSAGAMSLESGLTTHSVLAIERGPNSLANSGSDFGGGGLGLPLRLLRVSVGTQTSRSDWVDLVSWSHPGPTSKSQQVDLVSLFPKHRVDLLSKNDQVDLVAQFLPSKFPPNLAENDLALLVNLEFYRSDLHVYECVHFAAHWEGLSGLPEVYEQLAPQPCVGETLHSSLPRDSELFVPEEGSSEKESEDAPKTSPPTPGKHGLEQTGEEKVMVTVPDKNPPCPCCGTRVNSVLNLIEHLKVSHGKRGVCFRCAKCGKENSNYHSVVCHFPKCRGPETEKAPAGEWICEVCNRDFTTKIGLGQHKRLAHPAVRNQERIVASQPKETSNRGARKRCWTKEEEELLIRLEAQFEGNKNINKLIAEHITTKTAKQISDKRRLLSRKPAEEPREEPGTCHHTRRAAASLRTEPEMSHHAQAEDRDNGPGRRPLPGRAAAGGRTMDEIRRHPDKGNGQQRPTKQKSEEQLQAYYKKTLEERLSAGALNTFPRAFKQVMEGRDIKLVINQTAQDCFGCLESISQIRTATRDKKDTVTREKHPKKPFQKWMKDRAIKKGNYLRFQRLFYLDRGKLAKIILDDIECLSCDIPLSEIYSVFKTRWETTGSFKSLGDFKTYGKADNTAFRELITAKEIEKNVQEMSKGSAPGPDGITLGDVVKMDPEFSRTMEIFNLWLTTGKIPDMVRGCRTVLIPKSSKPDRLKDINNWRPITIGSILLRLFSRIVTARLSKACPLNPRQRGFIRAAGCSENLKLLQTIIWSAKREHRPLGVVFVDIAKAFDTVSHQHIIHVLQQREVDPHIVGLVSNMYENISTYITTKRNTHTDKIQIRVGVKQGDPMSPLLFNLAMDPLLCKLEESGKGYHRGQSSITAMAFADDLVLLSDSWENMNTNISILETFCNLTGLKTQGQKCHGFYIKPTKDSYTINDCAAWTINGTPLNMIDPGESEKYLGLRFDPWIGIARSGLSTKLDFWLQRIDQAPLKPLQKTDILKTYTIPRLIYIADHSEVKTALLETLDQKIRTAVKEWLHLPPCTCDAILYSSTRDGGLGITKLAGLIPSVQARRLHRIAQSSDDTMKCFMEKEKMEQLHKKLWIQARGDRENIPSIWEAPPSSEPPNNVSTNSEWEAPTQKDKFPKPCNWRKNEFKKWTKLASQGRGIVNFERDKISNHWIQYYRRIPHRKLLTALQLRANVYPTREFLARGRQDQYIKACRHCDADIESCAHIIGNCPVTQDARIKRHNYICELLLEEAKKKDWVVFKEPHIRDSNKELYKPDLIFVKDARALVVDVTVRYEAAKSSLEEAAAEKVRKYKHLETEVRHLTNAKDVTFVGFPLGARGKWHQDNFKLLTELGLSKSRQVKMAETFSTVALFSSVDIVHMFASRARKSMVM

SEQ ID NO: 8 - protein, 291 aa, synthetic construct
MSKSWGKFIEEEEAEMASRRNLMIVDGTNLGFRFKHNNSKKPFASSYVSTIQSLAKSYSARTTIVLGDKGKSVFRLEHLPEYKGNRDEKYAQRTEEEKALDEQFFEYLKDAFELCKTTFPTFTIRGVEADDMAAYIVKLIGHLYDHVWLISTDGDWDTLLTDKVSRFSFTTRREYHLRDMYEHHNVDDVEQFISLKAIMGDLGDNIRGVEGIGAKRGYNIIREFGNVLDIIDQLPLPGKQKYIQNLNASEELLFRNLILVDLPTYCVDAIAAVGQDVLDKFTKDILEIAEQ

SEQ ID NO: 9 - protein, 64 aa, synthetic construct
MVTVKFKYKGEELEVDISKIKKVWRVGKMISFTYDDNGKTGRGAVSEKDAPKELLQMLEKSGKK

SEQ ID NO: 10 - protein, 100 aa, synthetic construct
MPKRKVSSAEGAAKEEPKRRSARLSAKPPAKVEAKPKKAAAKDKSSDKKVQTKGKRGAKGKQAEVANQETKEDLPAENGETKTEESPASDEAGEKEAKSD

SEQ ID NO: 11 - protein, 195 aa, synthetic construct
DILAEAHGTRPDLTDQPLPDADHTWYTDGSSLLQEGQRKAGAAVTTETEVIWAKALPAGTSAQRAELIALTQALKMAEGKKLNVYTDSRYAFATAHIHGEIYRRRGWLTSEGKEIKNKDEILALLKALFLPKRLSIIHCPGHQKGHSAEARGNRMADQAARKAAITETPDTSTLLIENSSPSGGSKRTADGSEFE

SEQ ID NO: 12 - protein, 1374 aa, synthetic construct
MPKRKVSSAEGAAKEEPKRRSARLSAKPPAKVEAKPKKAAAKDKSSDKKVQTKGKRGAKGKQAEVANQETKEDLPAENGETKTEESPASDEAGEKEAKSDVMVTVPDKNPPCPCCGTRVNSVLNLIEHLKVSHGKRGVCFRCAKCGKENSNYHSVVCHFPKCRGPETEKAPAGEWICEVCNRDFTTKIGLGQHKRLAHPAVRNQERIVASQPKETSNRGAHKRCWTKEEEELLIRLEAQFEGNKNINKLIAEHITTKTAKQISDKRRLLSRKPAEEPREEPGTCHHTRRAAASLRTEPEMSHHAQAEDRDNGGGMPKRKVSSAEGAAKEEPKRRSARLSAKPPAKVEAKPKKAAAKDKSSDKKVQTKGKRGAKGKQAEVANQETKEDLPAENGETKTEESPASDEAGEKEAKSDGGPGRRPLPGRAAAGGRTMDEIRRHPDKGNGQQRPTKQKSEEQLQAYYKKTLEERLSAGALNTFPRAFKQVMEGRDIKLVINQTAQDCFGCLESISQIRTATRDKKDTVTREKHPKKPFQKWMKDRAIKKGNYLRFQRLFYLDRGKLAKIILDDIECLSCDIPLSEIYSVFKTRWETTGSFKSLGDFKTYGKADNTAFRELITAKEIEKNVQEMSKGSAPGPDGITLGDVVKMDPEFSRTMEIFNLWLTTGKIPDMVRGCRTVLIPKSSKPDRLKDINNWRPITIGSILLRLFSRIVTARLSKACPLNPRQRGFIRAAGCSENLKLLQTIIWSAKREHRPLGVVFVDIAKAFDTVSHQHIIHALQQREVDPHIVGLVSNMYENISTYITTKRNTHTDKIQIRVGVKQGDPMSPLLFNLAMDPLLCKLEESGKGYHRGQSSITAMAFADDLVLLSDSWENMNTNISILETFCNLTGLKTQGQKCHGFYIKPTKDSYTINDCAAWTINGTPLNMIDPGESEKYLGLQFDPWIGIARSGLSTKLDFWLQRIDQAPLKPLQKTDILKTYTIPRLIYIADHSEVKTALLETLDQKIRTAVKEWLHLPPCTCDAILYSSTRDGGLGITKLAGLIPSVQARRLHRIAQSSDDTMKCFMEKEKMEQLHKKLWIQAGGDRENIPSIWEAPPSSEPPNNVSTNSEWEAPTQKDKFPKPCNWRKNEFKKWTKLASQGRGIVNFERDKISNHWIQYYRRIPHRKLLTALQLRANVYPTREFLARGRQDQYIKACRHCDADIESCAHIIGNCPVTQDARIKRHNYICELLLEEAKKKDWVVFKEPHIRDSNKELYKPDLIFVKDARALVVDVTVRYEAAKSSLEEAAAEKVRKYKHLETEVRHLTNAKDVTFVGFPLGARGKWHQDNFKLLTELGLSKSRQVKMAETFSTVALFSSVDIVHMFASRARKSMVM

SEQ ID NO: 13 - protein, 1279 aa, synthetic construct
MASCPKPGPPVSAGAMSLESGLTTHSVLAIERGPNSLANSGSDFGGGGLGLPLRLLRVSVGTQTSRSDWVDLVSWSHPGPTSKSQQVDLVSLFPKHRVDLLSKNDQVDLVAQFLPSKFPPNLAENDLALLVNLEFYRSDLHVYECVHFAAHWEGLSGLPEVYEQLAPQPCVGETLHSSLPRDSELFVPEEGSSEKESEDAPKTSPPTPGKHGLEQTGEEKVMVTVPDKNPPCPCCGTRVNSVLNLIEHLKVSHGKRGVCFRCAKCGKENSNYHSVVCHFPKCRGPETEKAPAGEWICEVCNRDFTTKIGLGQHKRLAHPAVRNQERIVASQPKETSNRGAHKRCWTKEEEELLIRLEAQFEGNKNINKLIAEHITTKTAKQISDKRRLLVMEGRDIKLVINQTAQDCFGCLESISQIRTATRDKKDTVTREKHPKKPFQKWMKDRAIKKGNYLRFQRLFYLDRGKLAKIILDDIECLSCDIPLSEIYSVFKTRWETTGSFKSLGDFKTYGKADNTAFRELITAKEIEKNVQEMSKGSAPGPDGITLGDVVKMDPEFSRTMEIFNLWLTTGKIPDMVRGCRTVLIPKSSKPDRLKDINNWRPITIGSILLRLFSRIVTARLSKACPLNPRQRGFIRAAGCSENLKLLQTIIWSAKREHRPLGVVFVDIAKAFDTVSHQHIIHALQQREVDPHIVGLVSNMYENISTYITTKRNTHTDKIQIRVGVKQGDPMSPLLFNLAMDPLLCKLEESGKGYHRGQSSITAMAFADDLVLLSDSWENMNTNISILETFCNLTGLKTQGQKCHGFYIKPTKDSYTINDCAAWTINGTPLNMIDPGESEKYLGLQFDPWIGIARSGLSTKLDFWLQRIDQAPLKPLQKTDILKTYTIPRLIYIADHSEVKTALLETLDQKIRTAVKEWLHLPPCTCDAILYSSTRDGGLGITKLAGLIPSVQARRLHRIAQSSDDTMKCFMEKEKMEQLHKKLWIQAGGDRENIPSIWEAPPSSEPPNNVSTNSEWEAPTQKDKFPKPCNWRKNEFKKWTKLASQGRGIVNFERDKISNHWIQYYRRIPHRKLLTALQLRANVYPTREFLARGRQDQYIKACRHCDADIESCAHIIGNCPVTQDARIKRHNYICELLLEEAKKKDWVVFKEPHIRDSNKELYKPDLIFVKDARALVVDVTVRYEAAKSSLEEAAAEKVRKYKHLETEVRHLTNAKDVTFVGFPLGARGKWHQDNFKLLTELGLSKSRQVKMAETFSTVALFSSVDIVHMFASRARKSMVM

SEQ ID NO: 14 - protein, 22 aa, synthetic construct
DYKDHDGDYKDHDIDYKDDDDK

SEQ ID NO: 15 - RNA, 150 nt, synthetic construct
  source 1..150: mol_type = other RNA
gaatccgactgtttaattaaaacaaagcatcgcgaaggcccgcggcgggtgttgacgcgatgtgatttctgcccagtgctctgaatgtcaaagtgaagaaattcaatgaagcgcgggtaaacggcgggagtaactatgactctcttaagg

SEQ ID NO: 16 - RNA, 175 nt, synthetic construct
  source 1..175: mol_type = other RNA
gtctagttacaactgggcatcgctgcagagatcgcacctcctcgtggtcccgctggtagcccttcgaagggtgactaagtcgatctctgccccaggtacggagccgttgggactcaccagtccaacgtaactcctgcctaaattcggtgaaacaaattcctcggtaaaaagcccc

SEQ ID NO: 17 - RNA, 325 nt, synthetic construct
  source 1..325: mol_type = other RNA
ttcaggttatttagatgcttagtttttgtacctttcttgttttgtttaggattttgatagtgttagtatttttatatttttgtacgattgcataatgttcttttttatacagttctgttttaataaaatagacgatagctagagacgttagggcagccacaagccagttaggtagcggatagtaggtaggaacagacttttactatttcataacgcgtcaattaccacctgatttggaccaattcacgggatttgtccaaggtggacgggccacctttacttaacccggaaaaggaacatatataatttatgtgtgttcgataaa

SEQ ID NO: 18 - RNA, 150 nt, synthetic construct
  source 1..150: mol_type = other RNA
tagccaaatgcctcgtcatctaattagtgacgcgcatgaatggatgaacgagattcccactgtccctacctactatccagcgaaaccacagccaagggaacgggcttggcggaatcagcggggaaagaagaccctgttgagcttgactct

SEQ ID NO: 19 - RNA, 100 nt, synthetic construct
  source 1..100: mol_type = other RNA
gttgacgcgatgtgatttctgcccagtgctctgaatgtcaaagtgaagaaattcaatgaagcgcgggtaaacggcgggagtaactatgactctcttaagg

SEQ ID NO: 20 - RNA, 100 nt, synthetic construct
  source 1..100: mol_type = other RNA
tagccaaatgcctcgtcatctaattagtgacgcgcatgaatggatgaacgagattcccactgtccctacctactatccagcgaaaccacagccaagggaa

SEQ ID NO: 21 - RNA, 50 nt, synthetic construct
  source 1..50: mol_type = other RNA
attcaatgaagcgcgggtaaacggcgggagtaactatgactctcttaagg

SEQ ID NO: 22 - RNA, 50 nt, synthetic construct
  source 1..50: mol_type = other RNA
tagccaaatgcctcgtcatctaattagtgacgcgcatgaatggatgaacg

SEQ ID NO: 23 - RNA, 20 nt, synthetic construct
  source 1..20: mol_type = other RNA
taactatgactctcttaagg

SEQ ID NO: 24 - RNA, 20 nt, synthetic construct
  source 1..20: mol_type = other RNA
tagccaaatgcctcgtcatc

SEQ ID NO: 25 - RNA, 10 nt, synthetic construct
  source 1..10: mol_type = other RNA
tctcttaagg

SEQ ID NO: 26 - RNA, 10 nt, synthetic construct
  source 1..10: mol_type = other RNA
tagccaaatg

SEQ ID NO: 27 - RNA, 168 nt, synthetic construct
  source 1..168: mol_type = other RNA
gtcaactgggcatcgctgcagagatcgcacctcctcgtggtcccgctggtagcccttcgaagggtgactaagtcgatctctgccccaggtacggagccgttgggactcaccagtccaacgtaactcctgcctaaattcggtgaaacaaattcctcggtaaaaagcccc

SEQ ID NO: 28 - RNA, 28 nt, synthetic construct
  source 1..28: mol_type = other RNA
ggcgggagtaactatgactctcttaagg

SEQ ID NO: 29 - RNA, 165 nt, synthetic construct
  source 1..165: mol_type = other RNA
aactgggcatcgctgcagagatcgcacctcctcgtggtcccgctggtagcccttcgaagggtgactaagtcgatctctgccccaggtacggagccgttgggactcaccagtccaacgtaactcctgcctaaattcggtgaaacaaattcctcggtaaaaagcccc

SEQ ID NO: 30 - RNA, 1314 nt, synthetic construct
  source 1..1314: mol_type = other RNA
gaacaaacgacccaacacccgtgcgttttattctgtctttttattgccgatcttacttgtacagctcgtccatgccgagagtgatcccggcggcggtcacgaactccagcaggaccatgtgatcgcgcttctcgttggggtctttgctcagggcggactgggtgctcaggtagtggttgtcgggcagcagcacggggccgtcgccgatgggggtgttctgctggtagtggtcggccagctgcacgctgccgtcctcgatgttgtggcggatcttgaagttcaccttgatgccgttcttctgcttgtcggccatgatatagacgttgtggctgttgtagttgtactccagcttgtgccccaggatgttgccgtcctccttgaagtcgatgcccttcagctcgatgcggttcaccagggtgtcgccctcgaacttcacctcggcgcgggtcttgtagttgccgtcgtccttgaagaagatggtgcgctcctggacgtagccttcgggcatggcggacttgaagaagtcgtgctgcttcatgtggtcggggtagcggctgaagcactgcacgccgtaggtcagggtggtcacgagggtgggccagggcacgggcagcttgccggtggtgcagatgaacttcagggtcagcttgccgtaggtggcatcgccctcgccctcgccggacacgctgaacttgtggccgtttacgtcgccgtccagctcgaccaggatgggcaccaccccggtgaacagctcctcgcccttgctcaccatggtggcgctagcggatctgacggttcactaaaccagctctgcttatatagacctcccaccgtacacgcctaccgcccatttgcgtcaatggggcggagttgttacgacattttggaaagtcccgttgattttggtgccaaaacaaactcccattgacgtcaatggggtggagacttggaaatccccgtgagtcaaaccgctatccacgcccattgatgtactgccaaaaccgcatcaccatggtaatagcgatgactaatacgtagatgtactgccaagtaggaaagtcccataaggtcatgtactgggcataatgccaggcgggccatttaccgtcattgacgtcaatagggggcgtacttggcatatgatacacttgatgtactgccaagtgggcagtttaccgtaaatactccacccattgacgtcaatggaaagtccctattggcgttactatgggaacatacgtcattattgacgtcaatgggcgggggtcgttgggcggtcagccaggcgggccatttaccgtaagttatgtaacg

SEQ ID NO: 31 - RNA, 109 nt, synthetic construct
  source 1..109: mol_type = other RNA
gtctagttacaactgggcatcgctcccaggtacggagccgttgggactcaccagtccaacgtaactcctgcctaaattcggtgaaacaaattcctcggtaaaaagcccc

SEQ ID NO: 32 - RNA, 81 nt, synthetic construct
  source 1..81: mol_type = other RNA
cacgggatttgtccaaggtggacgggccacctttacttaacccggaaaaggaacatatataatttatgtgtgttcgataaa

SEQ ID NO: 33 - RNA, 85 nt, synthetic construct
  source 1..85: mol_type = other RNA
cccaggtacggagccgttgggactcaccagtccaacgtaactcctgcctaaattcggtgaaacaaattcctcggtaaaaagcccc

SEQ ID NO: 34 - RNA, 65 nt, synthetic construct
  source 1..65: mol_type = other RNA
ggtggacgggccacctttacttaacccggaaaaggaacatatataatttatgtgtgttcgataaa

SEQ ID NO: 35 - RNA, 175 nt, synthetic construct
  source 1..175: mol_type = other RNA
gtctagttacaactgggcatcgctgcagagatcgcacctcctcgtggtcccgctggtagcccttcgaagggtgattaagtcgatctctgccccaggtacggagccgttgggactcaccagtccaacgtaactcctgcctaaattcggtgaaacaaattcctcggtaaaaagcccc

SEQ ID NO: 36 - skipped

SEQ ID NO: 37 - RNA, 129 nt, synthetic construct
  source 1..129: mol_type = other RNA
gtctagttacaactgggcatcgctgcagagatcgcacctcctcgtggtcccgctggtagcccttcgaagggtgactaagtcgatctctgccccaaattcggtgaaacaaattcctcggtaaaaagcccc

SEQ ID NO: 38 - protein, 1369 aa, synthetic construct
MASCPKPGPPVSAGAMSLESGLTTHSVLAIERGPNSLANSGSDFGGGGLGLPLRLLRVSVGTQTSRSDWVDLVSWSHPGPTSKSQQVDLVSLFPKHRVDLLSKNDQVDLVAQFLPSKFPPNLAENDLALLVNLEFYRSDLHVYECVHFAAHWEGLSGLPEVYEQLAPQPCVGETLHSSLPRDSELFVPEEGSSEKESEDAPKTSPPTPGKHGLEQTGEEKVMVTVPDKNPPCPCCGTRVNSVLNLIEHLKVSHGKRGVCFRCAKCGKENSNYHSVVCHFPKCRGPETEKAPAGEWICEVCNRDFTTKIGLGQHKRLAHPAVRNQERIVASQPKETSNRGAHKRCWTKEEEELLIRLEAQFEGNKNINKLIAEHITTKTAKQISDKRRLLSRKPAEEPREEPGTCHHTRRAAASLRTEPEMSHHAQAEDRDNGPGRRPLPGRAAAGGRTMDEIRRHPDKGNGQQRPTKQKSEEQLQAYYKKTLEERLSAGALNTFPRAFKQVMEGRDIKLVINQTAQDCFGCLESISQIRTATRDKKDTVTREKHPKKPFQKWMKDRAIKKGNYLRFQRLFYLDRGKLAKIILDDIECLSCDIPLSEIYSVFKTRWETTGSFKSLGDFKTYGKADNTAFRELITAKEIEKNVQEMSKGSAPGPDGITLGDVVKMDPEFSRTMEIFNLWLTTGKIPDMVRGCRTVLIPKSSKPDRLKDINNWRPITIGSILLRLFSRIVTARLSKACPLNPRQRGFIRAAGCSENLKLLQTIIWSAKREHRPLGVVFVDIAKAFDTVSHQHIIHALQQREVDPHIVGLVSNMYENISTYITTKRNTHTDKIQIRVGVKQGDPMSPLLFNLAMDPLLCKLEESGKGYHRGQSSITAMAFADDLVLLSDSWENMNTNISILETFCNLTGLKTQGQKCHGFYIKPTKDSYTINDCAAWTINGTPLNMIDPGESEKYLGLQFDPWIGIARSGLSTKLDFWLQRIDQAPLKPLQKTDILKTYTIPRLIYIADHSEVKTALLETLDQKIRTAVKEWLHLPPCTCDAILYSSTRDGGLGITKLAGLIPSVQARRLHRIAQSSDDTMKCFMEKEKMEQLHKKLWIQAGGSTNSEWEAPTQKDKFPKPCNWRKNEFKKWTKLASQGRGIVNFERDKISNHWIQYYRRIPHRKLLTALQLRANVYPTREFLARGRQDQYIKACRHCDADIESCAHIIGNCPVTQDARIKRHNYICELLLEEAKKKDWVVFKEPHIRDSNKELYKPDLIFVKDARALVVDVTVRYEAAKSSLEEAAAEKVRKYKHLETEVRHLTNAKDVTFVGFPLGARGKWHQDNFKLLTELGLSKSRQVKMAETFSTVALFSSVDIVHMFASRARKSMVM

SEQ ID NO: 39 - RNA, 142 nt, synthetic construct
  source 1..142: mol_type = other RNA
gtctagttacaactgggcatcgctgcagagatcgcacctcctcgtggtcccgctggtagcccttcgaagggtgactaagtcgatctctgccccaggtacggagccgttgggactcaccagtccaacgtaactcctgcctaaa

SEQ ID NO: 40 - protein, 1059 aa, synthetic construct
VMVTVPDKNPPCPCCGTRVNSVLNLIEHLKVSHGKRGVCFRCAKCGKENSNYHSVVCHFPKCRGPETEKAPAGEWICEVCNRDFTTKIGLGQHKRLAHPAVRNQERIVASQPKETSNRGAHKRCWTKEEEELLIRLEAQFEGNKNINKLIAEHITTKTAKQISDKRRLLVMEGRDIKLVINQTAQDCFGCLESISQIRTATRDKKDTVTREKHPKKPFQKWMKDRAIKKGNYLRFQRLFYLDRGKLAKIILDDIECLSCDIPLSEIYSVFKTRWETTGSFKSLGDFKTYGKADNTAFRELITAKEIEKNVQEMSKGSAPGPDGITLGDVVKMDPEFSRTMEIFNLWLTTGKIPDMVRGCRTVLIPKSSKPDRLKDINNWRPITIGSILLRLFSRIVTARLSKACPLNPRQRGFIRAAGCSENLKLLQTIIWSAKREHRPLGVVFVDIAKAFDTVSHQHIIHALQQREVDPHIVGLVSNMYENISTYITTKRNTHTDKIQIRVGVKQGDPMSPLLFNLAMDPLLCKLEESGKGYHRGQSSITAMAFADDLVLLSDSWENMNTNISILETFCNLTGLKTQGQKCHGFYIKPTKDSYTINDCAAWTINGTPLNMIDPGESEKYLGLQFDPWIGIARSGLSTKLDFWLQRIDQAPLKPLQKTDILKTYTIPRLIYIADHSEVKTALLETLDQKIRTAVKEWLHLPPCTCDAILYSSTRDGGLGITKLAGLIPSVQARRLHRIAQSSDDTMKCFMEKEKMEQLHKKLWIQAGGDRENIPSIWEAPPSSEPPNNVSTNSEWEAPTQKDKFPKPCNWRKNEFKKWTKLASQGRGIVNFERDKISNHWIQYYRRIPHRKLLTALQLRANVYPTREFLARGRQDQYIKACRHCDADIESCAHIIGNCPVTQDARIKRHNYICELLLEEAKKKDWVVFKEPHIRDSNKELYKPDLIFVKDARALVVDVTVRYEAAKSSLEEAAAEKVRKYKHLETEVRHLTNAKDVTFVGFPLGARGKWHQDNFKLLTELGLSKSRQVKMAETFSTVALFSSVDIVHMFASRARKSMVM

SEQ ID NO: 41 - RNA, 36 nt, synthetic construct
  source 1..36: mol_type = other RNA
aaattcggtgaaacaaattcctcggtaaaaagcccc

SEQ ID NO: 42 - protein, 1514 aa, synthetic construct
MPKRKVSSAEGAAKEEPKRRSARLSAKPPAKVEAKPKKAAAKDKSSDKKVQTKGKRGAKGKQAEVANQETKEDLPAENGETKTEESPASDEAGEKEAKSDTSKSQQVDLVSLFPKHRVDLLSKNDQVDLVAQFLPSKFPPNLAENDLALLVNLEFYRSDLHVYECVHFAAHWEGLSGLPEVYEQLAPQPCVGETLHSSLPRDSELFVPEEGSSEKESEDAPKTSPPTPGKHGLEQTGEEKVMVTVPDKNPPCPCCGTRVNSVLNLIEHLKVSHGKRGVCFRCAKCGKENSNYHSVVCHFPKCRGPETEKAPAGEWICEVCNRDFTTKIGLGQHKRLAHPAVRNQERIVASQPKETSNRGAHKRCWTKEEEELLIRLEAQFEGNKNINKLIAEHITTKTAKQISDKRRLLSRKPAEEPREEPGTCHHTRRAAASLRTEPEMSHHAQAEDRDNGGGMPKRKVSSAEGAAKEEPKRRSARLSAKPPAKVEAKPKKAAAKDKSSDKKVQTKGKRGAKGKQAEVANQETKEDLPAENGETKTEESPASDEAGEKEAKSDGGPGRRPLPGRAAAGGRTMDEIRRHPDKGNGQQRPTKQKSEEQLQAYYKKTLEERLSAGALNTFPRAFKQVMEGRDIKLVINQTAQDCFGCLESISQIRTATRDKKDTVTREKHPKKPFQKWMKDRAIKKGNYLRFQRLFYLDRGKLAKIILDDIECLSCDIPLSEIYSVFKTRWETTGSFKSLGDFKTYGKADNTAFRELITAKEIEKNVQEMSKGSAPGPDGITLGDVVKMDPEFSRTMEIFNLWLTTGKIPDMVRGCRTVLIPKSSKPDRLKDINNWRPITIGSILLRLFSRIVTARLSKACPLNPRQRGFIRAAGCSENLKLLQTIIWSAKREHRPLGVVFVDIAKAFDTVSHQHIIHVLQQREVDPHIVGLVSNMYENISTYITTKRNTHTDKIQIRVGVKQGDPMSPLLFNLAMDPLLCKLEESGKGYHRGQSSITAMAFADDLVLLSDSWENMNTNISILETFCNLTGLKTQGQKCHGFYIKPTKDSYTINDCAAWTINGTPLNMIDPGESEKYLGLRFDPWIGIARSGLSTKLDFWLQRIDQAPLKPLQKTDILKTYTIPRLIYIADHSEVKTALLETLDQKIRTAVKEWLHLPPCTCDAILYSSTRDGGLGITKLAGLIPSVQARRLHRIAQSSDDTMKCFMEKEKMEQLHKKLWIQARGDRENIPSIWEAPPSSEPPNNVSTNSEWEAPTQKDKFPKPCNWRKNEFKKWTKLASQGRGIVNFERDKISNHWIQYYRRIPHRKLLTALQLRANVYPTREFLARGRQDQYIKACRHCDADIESCAHIIGNCPVTQDARIKRHNYICELLLEEAKKKDWVVFKEPHIRDSNKELYKPDLIFVKDARALVVDVTVRYEAAKSSLEEAAAEKVRKYKHLETEVRHLTNAKDVTFVGFPLGARGKWHQDNFKLLTELGLSKSRQVKMAETFSTVALFSSVDIVHMFASRARKSMVM

SEQ ID NO: 43 - protein, 1404 aa, synthetic construct
MPKRKVSSAEGAAKEEPKRRSARLSAKPPAKVEAKPKKAAAKDKSSDKKVQTKGKRGAKGKQAEVANQETKEDLPAENGETKTEESPASDEAGEKEAKSDGSSEKESEDAPKTSPPTPGKHGLEQTGEEKVMVTVPDKNPPCPCCGTRVNSVLNLIEHLKVSHGKRGVCFRCAKCGKENSNYHSVVCHFPKCRGPETEKAPAGEWICEVCNRDFTTKIGLGQHKRLAHPAVRNQERIVASQPKETSNRGAHKRCWTKEEEELLIRLEAQFEGNKNINKLIAEHITTKTAKQISDKRRLLSRKPAEEPREEPGTCHHTRRAAASLRTEPEMSHHAQAEDRDNGGGMPKRKVSSAEGAAKEEPKRRSARLSAKPPAKVEAKPKKAAAKDKSSDKKVQTKGKRGAKGKQAEVANQETKEDLPAENGETKTEESPASDEAGEKEAKSDGGPGRRPLPGRAAAGGRTMDEIRRHPDKGNGQQRPTKQKSEEQLQAYYKKTLEERLSAGALNTFPRAFKQVMEGRDIKLVINQTAQDCFGCLESISQIRTATRDKKDTVTREKHPKKPFQKWMKDRAIKKGNYLRFQRLFYLDRGKLAKIILDDIECLSCDIPLSEIYSVFKTRWETTGSFKSLGDFKTYGKADNTAFRELITAKEIEKNVQEMSKGSAPGPDGITLGDVVKMDPEFSRTMEIFNLWLTTGKIPDMVRGCRTVLIPKSSKPDRLKDINNWRPITIGSILLRLFSRIVTARLSKACPLNPRQRGFIRAAGCSENLKLLQTIIWSAKREHRPLGVVFVDIAKAFDTVSHQHIIHVLQQREVDPHIVGLVSNMYENISTYITTKRNTHTDKIQIRVGVKQGDPMSPLLFNLAMDPLLCKLEESGKGYHRGQSSITAMAFADDLVLLSDSWENMNTNISILETFCNLTGLKTQGQKCHGFYIKPTKDSYTINDCAAWTINGTPLNMIDPGESEKYLGLRFDPWIGIARSGLSTKLDFWLQRIDQAPLKPLQKTDILKTYTIPRLIYIADHSEVKTALLETLDQKIRTAVKEWLHLPPCTCDAILYSSTRDGGLGITKLAGLIPSVQARRLHRIAQSSDDTMKCFMEKEKMEQLHKKLWIQARGDRENIPSIWEAPPSSEPPNNVSTNSEWEAPTQKDKFPKPCNWRKNEFKKWTKLASQGRGIVNFERDKISNHWIQYYRRIPHRKLLTALQLRANVYPTREFLARGRQDQYIKACRHCDADIESCAHIIGNCPVTQDARIKRHNYICELLLEEAKKKDWVVFKEPHIRDSNKELYKPDLIFVKDARALVVDVTVRYEAAKSSLEEAAAEKVRKYKHLETEVRHLTNAKDVTFVGFPLGARGKWHQDNFKLLTELGLSKSRQVKMAETFSTVALFSSVDIVHMFASRARKSMVM

SEQ ID NO: 44 - RNA, 93 nt, synthetic construct
  source 1..93: mol_type = other RNA
tttggaccaattcacgggatttgtccaaggtggacgggccacctttacttaacccggaaaaggaacatatataatttatgtgtgttcgataaa

SEQ ID NO: 45 - protein, 1374 aa, synthetic construct
MPKRKVSSAEGAAKEEPKRRSARLSAKPPAKVEAKPKKAAAKDKSSDKKVQTKGKRGAKGKQAEVANQETKEDLPAENGETKTEESPASDEAGEKEAKSDVMVTVPDKNPPCPCCGTRVNSVLNLIEHLKVSHGKRGVCFRCAKCGKENSNYHSVVCHFPKCRGPETEKAPAGEWICEVCNRDFTTKIGLGQHKRLAHPAVRNQERIVASQPKETSNRGAHKRCWTKEEEELLIRLEAQFEGNKNINKLIAEHITTKTAKQISDKRRLLSRKPAEEPREEPGTCHHTRRAAASLRTEPEMSHHAQAEDRDNGGGMPKRKVSSAEGAAKEEPKRRSARLSAKPPAKVEAKPKKAAAKDKSSDKKVQTKGKRGAKGKQAEVANQETKEDLPAENGETKTEESPASDEAGEKEAKSDGGPGRRPLPGRAAAGGRTMDEIRRHPDKGNGQQRPTKQKSEEQLQAYYKKTLEERLSAGALNTFPRAFKQVMEGRDIKLVINQTAQDCFGCLESISQIRTATRDKKDTVTREKHPKKPFQKWMKDRAIKKGNYLRFQRLFYLDRGKLAKIILDDIECLSCDIPLSEIYSVFKTRWETTGSFKSLGDFKTYGKADNTAFRELITAKEIEKNVQEMSKGSAPGPDGITLGDVVKMDPEFSRTMEIFNLWLTTGKIPDMVRGCRTVLIPKSSKPDRLKDINNWRPITIGSILLRLFSRIVTARLSKACPLNPRQRGFIRAAGCSENLKLLQTIIWSAKREHRPLGVVFVDIAKAFDTVSHQHIIHVLQQREVDPHIVGLVSNMYENISTYITTKRNTHTDKIQIRVGVKQGDPMSPLLFNLAMDPLLCKLEESGKGYHRGQSSITAMAFADDLVLLSDSWENMNTNISILETFCNLTGLKTQGQKCHGFYIKPTKDSYTINDCAAWTINGTPLNMIDPGESEKYLGLRFDPWIGIARSGLSTKLDFWLQRIDQAPLKPLQKTDILKTYTIPRLIYIADHSEVKTALLETLDQKIRTAVKEWLHLPPCTCDAILYSSTRDGGLGITKLAGLIPSVQARRLHRIAQSSDDTMKCFMEKEKMEQLHKKLWIQARGDRENIPSIWEAPPSSEPPNNVSTNSEWEAPTQKDKFPKPCNWRKNEFKKWTKLASQGRGIVNFERDKISNHWIQYYRRIPHRKLLTALQLRANVYPTREFLARGRQDQYIKACRHCDADIESCAHIIGNCPVTQDARIKRHNYICELLLEEAKKKDWVVFKEPHIRDSNKELYKPDLIFVKDARALVVDVTVRYEAAKSSLEEAAAEKVRKYKHLETEVRHLTNAKDVTFVGFPLGARGKWHQDNFKLLTELGLSKSRQVKMAETFSTVALFSSVDIVHMFASRARKSMVM

SEQ ID NO: 46 - RNA, 81 nt, synthetic construct; identical to SEQ ID NO: 32
  source 1..81: mol_type = other RNA

SEQ ID NO: 47 - protein, 1310 aa, synthetic construct
TSKSQQVDLVSLFPKHRVDLLSKNDQVDLVAQFLPSKFPPNLAENDLALLVNLEFYRSDLHVYECVHFAAHWEGLSGLPEVYEQLAPQPCVGETLHSSLPRDSELFVPEEGSSEKESEDAPKTSPPTPGKHGLEQTGEEKVMVTVPDKNPPCPCCGTRVNSVLNLIEHLKVSHGKRGVCFRCAKCGKENSNYHSVVCHFPKCRGPETEKAPAGEWICEVCNRDFTTKIGLGQHKRLAHPAVRNQERIVASQPKETSNRGAHKRCWTKEEEELLIRLEAQFEGNKNINKLIAEHITTKTAKQISDKRRLLSRKPAEEPREEPGTCHHTRRAAASLRTEPEMSHHAQAEDRDNGPGRRPLPGRAAAGGRTMDEIRRHPDKGNGQQRPTKQKSEEQLQAYYKKTLEERLSAGALNTFPRAFKQVMEGRDIKLVINQTAQDCFGCLESISQIRTATRDKKDTVTREKHPKKPFQKWMKDRAIKKGNYLRFQRLFYLDRGKLAKIILDDIECLSCDIPLSEIYSVFKTRWETTGSFKSLGDFKTYGKADNTAFRELITAKEIEKNVQEMSKGSAPGPDGITLGDVVKMDPEFSRTMEIFNLWLTTGKIPDMVRGCRTVLIPKSSKPDRLKDINNWRPITIGSILLRLFSRIVTARLSKACPLNPRQRGFIRAAGCSENLKLLQTIIWSAKREHRPLGVVFVDIAKAFDTVSHQHIIHALQQREVDPHIVGLVSNMYENISTYITTKRNTHTDKIQIRVGVKQGDPMSPLLFNLAMDPLLCKLEESGKGYHRGQSSITAMAFADDLVLLSDSWENMNTNISILETFCNLTGLKTQGQKCHGFYIKPTKDSYTINDCAAWTINGTPLNMIDPGESEKYLGLQFDPWIGIARSGLSTKLDFWLQRIDQAPLKPLQKTDILKTYTIPRLIYIADHSEVKTALLETLDQKIRTAVKEWLHLPPCTCDAILYSSTRDGGLGITKLAGLIPSVQARRLHRIAQSSDDTMKCFMEKEKMEQLHKKLWIQAGGDRENIPSIWEAPPSSEPPNNVSTNSEWEAPTQKDKFPKPCNWRKNEFKKWTKLASQGRGIVNFERDKISNHWIQYYRRIPHRKLLTALQLRANVYPTREFLARGRQDQYIKACRHCDADIESCAHIIGNCPVTQDARIKRHNYICELLLEEAKKKDWVVFKEPHIRDSNKELYKPDLIFVKDARALVVDVTVRYEAAKSSLEEAAAEKVRKYKHLETEVRHLTNAKDVTFVGFPLGARGKWHQDNFKLLTELGLSKSRQVKMAETFSTVALFSSVDIVHMFASRARKSMVM

SEQ ID NO: 48 - RNA, 133 nt, synthetic construct
  source 1..133: mol_type = other RNA
ttcaggttatttagatgcgaaagcgtcaattaccacctgatttggaccaattcacgggatttgtccaaggtggacgggccacctttacttaacccggaaaaggaacatatataatttatgtgtgttcgataaa

SEQ ID NO: 49 - protein, 1200 aa, synthetic construct
GSSEKESEDAPKTSPPTPGKHGLEQTGEEKVMVTVPDKNPPCPCCGTRVNSVLNLIEHLKVSHGKRGVCFRCAKCGKENSNYHSVVCHFPKCRGPETEKAPAGEWICEVCNRDFTTKIGLGQHKRLAHPAVRNQERIVASQPKETSNRGAHKRCWTKEEEELLIRLEAQFEGNKNINKLIAEHITTKTAKQISDKRRLLSRKPAEEPREEPGTCHHTRRAAASLRTEPEMSHHAQAEDRDNGPGRRPLPGRAAAGGRTMDEIRRHPDKGNGQQRPTKQKSEEQLQAYYKKTLEERLSAGALNTFPRAFKQVMEGRDIKLVINQTAQDCFGCLESISQIRTATRDKKDTVTREKHPKKPFQKWMKDRAIKKGNYLRFQRLFYLDRGKLAKIILDDIECLSCDIPLSEIYSVFKTRWETTGSFKSLGDFKTYGKADNTAFRELITAKEIEKNVQEMSKGSAPGPDGITLGDVVKMDPEFSRTMEIFNLWLTTGKIPDMVRGCRTVLIPKSSKPDRLKDINNWRPITIGSILLRLFSRIVTARLSKACPLNPRQRGFIRAAGCSENLKLLQTIIWSAKREHRPLGVVFVDIAKAFDTVSHQHIIHALQQREVDPHIVGLVSNMYENISTYITTKRNTHTDKIQIRVGVKQGDPMSPLLFNLAMDPLLCKLEESGKGYHRGQSSITAMAFADDLVLLSDSWENMNTNISILETFCNLTGLKTQGQKCHGFYIKPTKDSYTINDCAAWTINGTPLNMIDPGESEKYLGLQFDPWIGIARSGLSTKLDFWLQRIDQAPLKPLQKTDILKTYTIPRLIYIADHSEVKTALLETLDQKIRTAVKEWLHLPPCTCDAILYSSTRDGGLGITKLAGLIPSVQARRLHRIAQSSDDTMKCFMEKEKMEQLHKKLWIQAGGDRENIPSIWEAPPSSEPPNNVSTNSEWEAPTQKDKFPKPCNWRKNEFKKWTKLASQGRGIVNFERDKISNHWIQYYRRIPHRKLLTALQLRANVYPTREFLARGRQDQYIKACRHCDADIESCAHIIGNCPVTQDARIKRHNYICELLLEEAKKKDWVVFKEPHIRDSNKELYKPDLIFVKDARALVVDVTVRYEAAKSSLEEAAAEKVRKYKHLETEVRHLTNAKDVTFVGFPLGARGKWHQDNFKLLTELGLSKSRQVKMAETFSTVALFSSVDIVHMFASRARKSMVM

SEQ ID NO: 50 - RNA, 283 nt, synthetic construct
  source 1..283: mol_type = other RNA
ttcaggttatttagatgcttagtttttgtacctttcttgttttgtttaggattttgatagtgttagtatttttatatttttgtacgattgcataatgttcttttttatacagttctgttttaataaaatagacgatagctagagacgttagggcagccacaagccagttaggtagcggatagtaggtaggaacagacttttactatttcataacgcgtcaattaccacctgatttggaccaattcagaaaaggaacatatataatttatgtgtgttcgataaa

SEQ ID NO: 51 - protein, 1170 aa, synthetic construct
VMVTVPDKNPPCPCCGTRVNSVLNLIEHLKVSHGKRGVCFRCAKCGKENSNYHSVVCHFPKCRGPETEKAPAGEWICEVCNRDFTTKIGLGQHKRLAHPAVRNQERIVASQPKETSNRGAHKRCWTKEEEELLIRLEAQFEGNKNINKLIAEHITTKTAKQISDKRRLLSRKPAEEPREEPGTCHHTRRAAASLRTEPEMSHHAQAEDRDNGPGRRPLPGRAAAGGRTMDEIRRHPDKGNGQQRPTKQKSEEQLQAYYKKTLEERLSAGALNTFPRAFKQVMEGRDIKLVINQTAQDCFGCLESISQIRTATRDKKDTVTREKHPKKPFQKWMKDRAIKKGNYLRFQRLFYLDRGKLAKIILDDIECLSCDIPLSEIYSVFKTRWETTGSFKSLGDFKTYGKADNTAFRELITAKEIEKNVQEMSKGSAPGPDGITLGDVVKMDPEFSRTMEIFNLWLTTGKIPDMVRGCRTVLIPKSSKPDRLKDINNWRPITIGSILLRLFSRIVTARLSKACPLNPRQRGFIRAAGCSENLKLLQTIIWSAKREHRPLGVVFVDIAKAFDTVSHQHIIHALQQREVDPHIVGLVSNMYENISTYITTKRNTHTDKIQIRVGVKQGDPMSPLLFNLAMDPLLCKLEESGKGYHRGQSSITAMAFADDLVLLSDSWENMNTNISILETFCNLTGLKTQGQKCHGFYIKPTKDSYTINDCAAWTINGTPLNMIDPGESEKYLGLQFDPWIGIARSGLSTKLDFWLQRIDQAPLKPLQKTDILKTYTIPRLIYIADHSEVKTALLETLDQKIRTAVKEWLHLPPCTCDAILYSSTRDGGLGITKLAGLIPSVQARRLHRIAQSSDDTMKCFMEKEKMEQLHKKLWIQAGGDRENIPSIWEAPPSSEPPNNVSTNSEWEAPTQKDKFPKPCNWRKNEFKKWTKLASQGRGIVNFERDKISNHWIQYYRRIPHRKLLTALQLRANVYPTREFLARGRQDQYIKACRHCDADIESCAHIIGNCPVTQDARIKRHNYICELLLEEAKKKDWVVFKEPHIRDSNKELYKPDLIFVKDARALVVDVTVRYEAAKSSLEEAAAEKVRKYKHLETEVRHLTNAKDVTFVGFPLGARGKWHQDNFKLLTELGLSKSRQVKMAETFSTVALFSSVDIVHMFASRARKSMVM

SEQ ID NO: 52 - RNA, 291 nt, synthetic construct
  source 1..291: mol_type = other RNA
ttcaggttatttagatgcttagtttttgtacctttcttgttttgtttaggattttgatagtgttagtatttttatatttttgtacgattgcataatgttcttttttatacagttctgttttaataaaatagacgatagctagagacgttagggcagccacaagccagttaggtagcggatagtaggtaggaacagacttttactatttcataacgcgtcaattaccacctgatttggaccaattcacgggatttgtccaaggtggacgggccacctttacttaacccggaa

SEQ ID NO: 53 - protein, 461 aa, synthetic construct
MQRVNMIMAESPGLITICLLGYLLSAECTVFLDHENANKILNRPKRYNSGKLEEFVQGNLERECMEEKCSFEEAREVFENTERTTEFWKQYVDGDQCESNPCLNGGSCKDDINSYECWCPFGFEGKNCELDVTCNIKNGRCEQFCKNSADNKVVCSCTEGYRLAENQKSCEPAVPFPCGRVSVSQTSKLTRAETVFPDVDYVNSTEAETILDNITQSTQSFNDFTRVVGGEDAKPGQFPWQVVLNGKVDAFCGGSIVNEKWIVTAAHCVETGVKITVVAGEHNIEETEHTEQKRNVIRIIPHHNYNAAINKYNHDIALLELDEPLVLNSYVTPICIADKEYTNIFLKFGSGYVSGWGRVFHKGRSALVLQYLRVPLVDRATCLLSTKFTIYNNMFCAGFHEGGRDSCQGDSGGPHVTEVEGTSFLTGIISWGEECAMKGKYGIYTKVSRYVNWIKEKTKLT

SEQ ID NO: 54 - RNA, 37 nt, synthetic construct
  source 1..37: mol_type = other RNA
gaaaaggaacatatataatttatgtgtgttcgataaa

SEQ ID NO: 55 - protein, 1783 aa, synthetic construct
SKSWGKFIEEEEAEMASRRNLMIVDGTNLGFRFKHNNSKKPFASSYVSTIQSLAKSYSARTTIVLGDKGKSVFRLEHLPEYKGNRDEKYAQRTEEEKALDEQFFEYLKDAFELCKTTFPTFTIRGVEADDMAAYIVKLIGHLYDHVWLISTDGDWDTLLTDKVSRFSFTTRREYHLRDMYEHHNVDDVEQFISLKAIMGDLGDNIRGVEGIGAKRGYNIIREFGNVLDIIDQLPLPGKQKYIQNLNASEELLFRNLILVDLPTYCVDAIAAVGQDVLDKFTKDILEIAEQASCPKPGPPVSAGAMSLESGLTTHSVLAIERGPNSLANSGSDFGGGGLGLPLRLLRVSVGTQTSRSDWVDLVSWSHPGPTSKSQQVDLVSLFPKHRVDLLSKNDQVDLVAQFLPSKFPPNLAENDLALLVNLEFYRSDLHVYECVHFAAHWEGLSGLPEVYEQLAPQPCVGETLHSSLPRDSELFVPEEGSSEKESEDAPKTSPPTPGKHGLEQTGEEKVMVTVPDKNPPCPCCGTRVNSVLNLIEHLKVSHGKRGVCFRCAKCGKENSNYHSVVCHFPKCRGPETEKAPAGEWICEVCNRDFTTKIGLGQHKRLAHPAVRNQERIVASQPKETSNRGAHKRCWTKEEEELLIRLEAQFEGNKNINKLIAEHITTKTAKQISDKRRLLSRKPAEEPREEPGTCHHTRRAAASLRTEPEMSHHAQAEDRDNGGGMPKRKVSSAEGAAKEEPKRRSARLSAKPPAKVEAKPKKAAAKDKSSDKKVQTKGKRGAKGKQAEVANQETKEDLPAENGETKTEESPASDEAGEKEAKSDGGPGRRPLPGRAAAGGRTMDEIRRHPDKGNGQQRPTKQKSEEQLQAYYKKTLEERLSAGALNTFPRAFKQVMEGRDIKLVINQTAQDCFGCLESISQIRTATRDKKDTVTREKHPKKPFQKWMKDRAIKKGNYLRFQRLFYLDRGKLAKIILDDIECLSCDIPLSEIYSVFKTRWETTGSFKSLGDFKTYGKADNTAFRELITAKEIEKNVQEMSKGSAPGPDGITLGDVVKMDPEFSRTMEIFNLWLTTGKIPDMVRGCRTVLIPKSSKPDRLKDINNWRPITIGSILLRLFSRIVTARLSKACPLNPRQRGFIRAAGCSENLKLLQTIIWSAKREHRPLGVVFVDIAKAFDTVSHQHIIHALQQREVDPHIVGLVSNMYENISTYITTKRNTHTDKIQIRVGVKQGDPMSPLLFNLAMDPLLCKLEESGKGYHRGQSSITAMAFADDLVLLSDSWENMNTNISILETFCNLTGLKTQGQKCHGFYIKPTKDSYTINDCAAWTINGTPLNMIDPGESEKYLGLQFDPWIGIARSGLSTKLDFWLQRIDQAPLKPLQKTDILKTYTIPRLIYIADHSEVKTALLETLDQKIRTAVKEWLHLPPCTCDAILYSSTRDGGLGITKLAGLIPSVQARRLHRIAQSSDDTMKCFMEKEKMEQLHKKLWIQAGGDRENIPSIWEAPPSSEPPNNVSTNSEWEAPTQKDKFPKPCNWRKNEFKKWTKLASQGRGIVNFERDKISNHWIQYYRRIPHRKLLTALQLRANVYPTREFLARGRQDQYIKACRHCDADIESCAHIIGNCPVTQDARIKRHNYICELLLEEAKKKDWVVFKEPHIRDSNKELYKPDLIFVKDARALVVDVTVRYEAAKSSLEEAAAEKVRKYKHLETEVRHLTNAKDVTFVGFPLGARGKWHQDNFKLLTELGLSKSRQVKMAETFSTVALFSSVDIVHMFASRARKSMVM

SEQ ID NO: 56 - protein, 1878 aa, synthetic construct
SKSWGKFIEEEEAEMASRRNLMIVDGTNLGFRFKHNNSKKPFASSYVSTIQSLAKSYSARTTIVLGDKGKSVFRLEHLPEYKGNRDEKYAQRTEEEKALDEQFFEYLKDAFELCKTTFPTFTIRGVEADDMAAYIVKLIGHLYDHVWLISTDGDWDTLLTDKVSRFSFTTRREYHLRDMYEHHNVDDVEQFISLKAIMGDLGDNIRGVEGIGAKRGYNIIREFGNVLDIIDQLPLPGKQKYIQNLNASEELLFRNLILVDLPTYCVDAIAAVGQDVLDKFTKDILEIAEQASCPKPGPPVSAGAMSLESGLTTHSVLAIERGPNSLANSGSDFGGGGLGLPLRLLRVSVGTQTSRSDWVDLVSWSHPGPTSKSQQVDLVSLFPKHRVDLLSKNDQVDLVAQFLPSKFPPNLAENDLALLVNLEFYRSDLHVYECVHFAAHWEGLSGLPEVYEQLAPQPCVGETLHSSLPRDSELFVPEEGSSEKESEDAPKTSPPTPGKHGLEQTGEEKVMVTVPDKNPPCPCCGTRVNSVLNLIEHLKVSHGKRGVCFRCAKCGKENSNYHSVVCHFPKCRGPETEKAPAGEWICEVCNRDFTTKIGLGQHKRLAHPAVRNQERIVASQPKETSNRGAHKRCWTKEEEELLIRLEAQFEGNKNINKLIAEHITTKTAKQISDKRRLLSRKPAEEPREEPGTCHHTRRAAASLRTEPEMSHHAQAEDRDNGGGDILAEAHGTRPDLTDQPLPDADHTWYTDGSSLLQEGQRKAGAAVTTETEVIWAKALPAGTSAQRAELIALTQALKMAEGKKLNVYTDSRYAFATAHIHGEIYRRRGWLTSEGKEIKNKDEILALLKALFLPKRLSIIHCPGHQKGHSAEARGNRMADQAARKAAITETPDTSTLLIENSSPSGGSKRTADGSEFEGGPGRRPLPGRAAAGGRTMDEIRRHPDKGNGQQRPTKQKSEEQLQAYYKKTLEERLSAGALNTFPRAFKQVMEGRDIKLVINQTAQDCFGCLESISQIRTATRDKKDTVTREKHPKKPFQKWMKDRAIKKGNYLRFQRLFYLDRGKLAKIILDDIECLSCDIPLSEIYSVFKTRWETTGSFKSLGDFKTYGKADNTAFRELITAKEIEKNVQEMSKGSAPGPDGITLGDVVKMDPEFSRTMEIFNLWLTTGKIPDMVRGCRTVLIPKSSKPDRLKDINNWRPITIGSILLRLFSRIVTARLSKACPLNPRQRGFIRAAGCSENLKLLQTIIWSAKREHRPLGVVFVDIAKAFDTVSHQHIIHALQQREVDPHIVGLVSNMYENISTYITTKRNTHTDKIQIRVGVKQGDPMSPLLFNLAMDPLLCKLEESGKGYHRGQSSITAMAFADDLVLLSDSWENMNTNISILETFCNLTGLKTQGQKCHGFYIKPTKDSYTINDCAAWTINGTPLNMIDPGESEKYLGLQFDPWIGIARSGLSTKLDFWLQRIDQAPLKPLQKTDILKTYTIPRLIYIADHSEVKTALLETLDQKIRTAVKEWLHLPPCTCDAILYSSTRDGGLGITKLAGLIPSVQARRLHRIAQSSDDTMKCFMEKEKMEQLHKKLWIQAGGDRENIPSIWEAPPSSEPPNNVSTNSEWEAPTQKDKFPKPCNWRKNEFKKWTKLASQGRGIVNFERDKISNHWIQYYRRIPHRKLLTALQLRANVYPTREFLARGRQDQYIKACRHCDADIESCAHIIGNCPVTQDARIKRHNYICELLLEEAKKKDWVVFKEPHIRDSNKELYKPDLIFVKDARALVVDVTVRYEAAKSSLEEAAAEKVRKYKHLETEVRHLTNAKDVTFVGFPLGARGKWHQDNFKLLTELGLSKSRQVKMAETFSTVALFSSVDIVHMFASRARKSMVM

SEQ ID NO: 57 - protein, 1556 aa, synthetic construct
VTVKFKYKGEELEVDISKIKKVWRVGKMISFTYDDNGKTGRGAVSEKDAPKELLQMLEKSGKKASCPKPGPPVSAGAMSLESGLTTHSVLAIERGPNSLANSGSDFGGGGLGLPLRLLRVSVGTQTSRSDWVDLVSWSHPGPTSKSQQVDLVSLFPKHRVDLLSKNDQVDLVAQFLPSKFPPNLAENDLALLVNLEFYRSDLHVYECVHFAAHWEGLSGLPEVYEQLAPQPCVGETLHSSLPRDSELFVPEEGSSEKESEDAPKTSPPTPGKHGLEQTGEEKVMVTVPDKNPPCPCCGTRVNSVLNLIEHLKVSHGKRGVCFRCAKCGKENSNYHSVVCHFPKCRGPETEKAPAGEWICEVCNRDFTTKIGLGQHKRLAHPAVRNQERIVASQPKETSNRGAHKRCWTKEEEELLIRLEAQFEGNKNINKLIAEHITTKTAKQISDKRRLLSRKPAEEPREEPGTCHHTRRAAASLRTEPEMSHHAQAEDRDNGGGMPKRKVSSAEGAAKEEPKRRSARLSAKPPAKVEAKPKKAAAKDKSSDKKVQTKGKRGAKGKQAEVANQETKEDLPAENGETKTEESPASDEAGEKEAKSDGGPGRRPLPGRAAAGGRTMDEIRRHPDKGNGQQRPTKQKSEEQLQAYYKKTLEERLSAGALNTFPRAFKQVMEGRDIKLVINQTAQDCFGCLESISQIRTATRDKKDTVTREKHPKKPFQKWMKDRAIKKGNYLRFQRLFYLDRGKLAKIILDDIECLSCDIPLSEIYSVFKTRWETTGSFKSLGDFKTYGKADNTAFRELITAKEIEKNVQEMSKGSAPGPDGITLGDVVKMDPEFSRTMEIFNLWLTTGKIPDMVRGCRTVLIPKSSKPDRLKDINNWRPITIGSILLRLFSRIVTARLSKACPLNPRQRGFIRAAGCSENLKLLQTIIWSAKREHRPLGVVFVDIAKAFDTVSHQHIIHALQQREVDPHIVGLVSNMYENISTYITTKRNTHTDKIQIRVGVKQGDPMSPLLFNLAMDPLLCKLEESGKGYHRGQSSITAMAFADDLVLLSDSWENMNTNISILETFCNLTGLKTQGQKCHGFYIKPTKDSYTINDCAAWTINGTPLNMIDPGESEKYLGLQFDPWIGIARSGLSTKLDFWLQRIDQAPLKPLQKTDILKTYTIPRLIYIADHSEVKTALLETLDQKIRTAVKEWLHLPPCTCDAILYSSTRDGGLGITKLAGLIPSVQARRLHRIAQSSDDTMKCFMEKEKMEQLHKKLWIQAGGDRENIPSIWEAPPSSEPPNNVSTNSEWEAPTQKDKFPKPCNWRKNEFKKWTKLASQGRGIVNFERDKISNHWIQYYRRIPHRKLLTALQLRANVYPTREFLARGRQDQYIKACRHCDADIESCAHIIGNCPVTQDARIKRHNYICELLLEEAKKKDWVVFKEPHIRDSNKELYKPDLIFVKDARALVVDVTVRYEAAKSSLEEAAAEKVRKYKHLETEVRHLTNAKDVTFVGFPLGARGKWHQDNFKLLTELGLSKSRQVKMAETFSTVALFSSVDIVHMFASRARKSMVM

SEQ ID NO: 58 - protein, 1651 aa, synthetic construct
VTVKFKYKGEELEVDISKIKKVWRVGKMISFTYDDNGKTGRGAVSEKDAPKELLQMLEKSGKKASCPKPGPPVSAGAMSLESGLTTHSVLAIERGPNSLANSGSDFGGGGLGLPLRLLRVSVGTQTSRSDWVDLVSWSHPGPTSKSQQVDLVSLFPKHRVDLLSKNDQVDLVAQFLPSKFPPNLAENDLALLVNLEFYRSDLHVYECVHFAAHWEGLSGLPEVYEQLAPQPCVGETLHSSLPRDSELFVPEEGSSEKESEDAPKTSPPTPGKHGLEQTGEEKVMVTVPDKNPPCPCCGTRVNSVLNLIEHLKVSHGKRGVCFRCAKCGKENSNYHSVVCHFPKCRGPETEKAPAGEWICEVCNRDFTTKIGLGQHKRLAHPAVRNQERIVASQPKETSNRGAHKRCWTKEEEELLIRLEAQFEGNKNINKLIAEHITTKTAKQISDKRRLLSRKPAEEPREEPGTCHHTRRAAASLRTEPEMSHHAQAEDRDNGGGDILAEAHGTRPDLTDQPLPDADHTWYTDGSSLLQEGQRKAGAAVTTETEVIWAKALPAGTSAQRAELIALTQALKMAEGKKLNVYTDSRYAFATAHIHGEIYRRRGWLTSEGKEIKNKDEILALLKALFLPKRLSIIHCPGHQKGHSAEARGNRMADQAARKAAITETPDTSTLLIENSSPSGGSKRTADGSEFEGGPGRRPLPGRAAAGGRTMDEIRRHPDKGNGQQRPTKQKSEEQLQAYYKKTLEERLSAGALNTFPRAFKQVMEGRDIKLVINQTAQDCFGCLESISQIRTATRDKKDTVTREKHPKKPFQKWMKDRAIKKGNYLRFQRLFYLDRGKLAKIILDDIECLSCDIPLSEIYSVFKTRWETTGSFKSLGDFKTYGKADNTAFRELITAKEIEKNVQEMSKGSAPGPDGITLGDVVKMDPEFSRTMEIFNLWLTTGKIPDMVRGCRTVLIPKSSKPDRLKDINNWRPITIGSILLRLFSRIVTARLSKACPLNPRQRGFIRAAGCSENLKLLQTIIWSAKREHRPLGVVFVDIAKAFDTVSHQHIIHALQQREVDPHIVGLVSNMYENISTYITTKRNTHTDKIQIRVGVKQGDPMSPLLFNLAMDPLLCKLEESGKGYHRGQSSITAMAFADDLVLLSDSWENMNTNISILETFCNLTGLKTQGQKCHGFYIKPTKDSYTINDCAAWTINGTPLNMIDPGESEKYLGLQFDPWIGIARSGLSTKLDFWLQRIDQAPLKPLQKTDILKTYTIPRLIYIADHSEVKTALLETLDQKIRTAVKEWLHLPPCTCDAILYSSTRDGGLGITKLAGLIPSVQARRLHRIAQSSDDTMKCFMEKEKMEQLHKKLWIQAGGDRENIPSIWEAPPSSEPPNNVSTNSEWEAPTQKDKFPKPCNWRKNEFKKWTKLASQGRGIVNFERDKISNHWIQYYRRIPHRKLLTALQLRANVYPTREFLARGRQDQYIKACRHCDADIESCAHIIGNCPVTQDARIKRHNYICELLLEEAKKKDWVVFKEPHIRDSNKELYKPDLIFVKDARALVVDVTVRYEAAKSSLEEAAAEKVRKYKHLETEVRHLTNAKDVTFVGFPLGARGKWHQDNFKLLTELGLSKSRQVKMAETFSTVALFSSVDIVHMFASRARKSMVM

SEQ ID NO: 59 - protein, 1593 aa, synthetic construct
MPKRKVSSAEGAAKEEPKRRSARLSAKPPAKVEAKPKKAAAKDKSSDKKVQTKGKRGAKGKQAEVANQETKEDLPAENGETKTEESPASDEAGEKEAKSDASCPKPGPPVSAGAMSLESGLTTHSVLAIERGPNSLANSGSDFGGGGLGLPLRLLRVSVGTQTSRSDWVDLVSWSHPGPTSKSQQVDLVSLFPKHRVDLLSKNDQVDLVAQFLPSKFPPNLAENDLALLVNLEFYRSDLHVYECVHFAAHWEGLSGLPEVYEQLAPQPCVGETLHSSLPRDSELFVPEEGSSEKESEDAPKTSPPTPGKHGLEQTGEEKVMVTVPDKNPPCPCCGTRVNSVLNLIEHLKVSHGKRGVCFRCAKCGKENSNYHSVVCHFPKCRGPETEKAPAGEWICEVCNRDFTTKIGLGQHKRLAHPAVRNQERIVASQPKETSNRGAHKRCWTKEEEELLIRLEAQFEGNKNINKLIAEHITTKTAKQISDKRRLLSRKPAEEPREEPGTCHHTRRAAASLRTEPEMSHHAQAEDRDNGGGMPKRKVSSAEGAAKEEPKRRSARLSAKPPAKVEAKPKKAAAKDKSSDKKVQTKGKRGAKGKQAEVANQETKEDLPAENGETKTEESPASDEAGEKEAKSDGGPGRRPLPGRAAAGGRTMDEIRRHPDKGNGQQRPTKQKSEEQLQAYYKKTLEERLSAGALNTFPRAFKQVMEGRDIKLVINQTAQDCFGCLESISQIRTATRDKKDTVTREKHPKKPFQKWMKDRAIKKGNYLRFQRLFYLDRGKLAKIILDDIECLSCDIPLSEIYSVFKTRWETTGSFKSLGDFKTYGKADNTAFRELITAKEIEKNVQEMSKGSAPGPDGITLGDVVKMDPEFSRTMEIFNLWLTTGKIPDMVRGCRTVLIPKSSKPDRLKDINNWRPITIGSILLRLFSRIVTARLSKACPLNPRQRGFIRAAGCSENLKLLQTIIWSAKREHRPLGVVFVDIAKAFDTVSHQHIIHALQQREVDPHIVGLVSNMYENISTYITTKRNTHTDKIQIRVGVKQGDPMSPLLFNLAMDPLLCKLEESGKGYHRGQSSITAMAFADDLVLLSDSWENMNTNISILETFCNLTGLKTQGQKCHGFYIKPTKDSYTINDCAAWTINGTPLNMIDPGESEKYLGLQFDPWIGIARSGLSTKLDFWLQRIDQAPLKPLQKTDILKTYTIPRLIYIADHSEVKTALLETLDQKIRTAVKEWLHLPPCTCDAILYSSTRDGGLGITKLAGLIPSVQARRLHRIAQSSDDTMKCFMEKEKMEQLHKKLWIQAGGDRENIPSIWEAPPSSEPPNNVSTNSEWEAPTQKDKFPKPCNWRKNEFKKWTKLASQGRGIVNFERDKISNHWIQYYRRIPHRKLLTALQLRANVYPTREFLARGRQDQYIKACRHCDADIESCAHIIGNCPVTQDARIKRHNYICELLLEEAKKKDWVVFKEPHIRDSNKELYKPDLIFVKDARALVVDVTVRYEAAKSSLEEAAAEKVRKYKHLETEVRHLTNAKDVTFVGFPLGARGKWHQDNFKLLTELGLSKSRQVKMAETFSTVALFSSVDIVHMFASRARKSMVM

SEQ ID NO: 60 - protein, 1697 aa, synthetic construct
MPKRKVSSAEGAAKEEPKRRSARLSAKPPAKVEAKPKKAAAKDKSSDKKVQTKGKRGAKGKQAEVANQETKEDLPAENGETKTEESPASDEAGEKEAKSDASCPKPGPPVSAGAMSLESGLTTHSVLAIERGPNSLANSGSDFGGGGLGLPLRLLRVSVGTQTSRSDWVDLVSWSHPGPTSKSQQVDLVSLFPKHRVDLLSKNDQVDLVAQFLPSKFPPNLAENDLALLVNLEFYRSDLHVYECVHFAAHWEGLSGLPEVYEQLAPQPCVGETLHSSLPRDSELFVPEEGSSEKESEDAPKTSPPTPGKHGLEQTGEEKVMVTVPDKNPPCPCCGTRVNSVLNLIEHLKVSHGKRGVCFRCAKCGKENSNYHSVVCHFPKCRGPETEKAPAGEWICEVCNRDFTTKIGLGQHKRLAHPAVRNQERIVASQPKETSNRGAHKRCWTKEEEELLIRLEAQFEGNKNINKLIAEHITTKTAKQISDKRRLLSRKPAEEPREEPGTCHHTRRAAASLRTEPEMSHHAQAEDRDNGGGMPKRKVSSAEGAAKEEPKRRSARLSAKPPAKVEAKPKKAAAKDKSSDKKVQTKGKRGAKGKQAEVANQETKEDLPAENGETKTEESPASDEAGEKEAKSDGGPGRRPLPGRAAAGGRTMDEIRRHPDKGNGQQRPTKQKSEEQLQAYYKKTLEERLSAGALNTFPRAFKQVMEGRDIKLVINQTAQDCFGCLESISQIRTATRDKKDTVTREKHPKKPFQKWMKDRAIKKGNYLRFQRLFYLDRGKLAKIILDDIECLSCDIPLSEIYSVFKTRWETTGSFKSLGDFKTYGKADNTAFRELITAKEIEKNVQEMSKGSAPGPDGITLGDVVKMDPEFSRTMEIFNLWLTTGKIPDMVRGCRTVLIPKSSKPDRLKDINNWRPITIGSILLRLFSRIVTARLSKACPLNPRQRGFIRAAGCSENLKLLQTIIWSAKREHRPLGVVFVDIAKAFDTVSHQHIIHALQQREVDPHIVGLVSNMYENISTYITTKRNTHTDKIQIRVGVKQGDPMSPLLFNLAMDPLLCKLEESGKGYHRGQSSITAMAFADDLVLLSDSWENMNTNISILETFCNLTGLKTQGQKCHGFYIKPTKDSYTINDCAAWTINGTPLNMIDPGESEKYLGLQFDPWIGIARSGLSTKLDFWLQRIDQAPLKPLQKTDILKTYTIPRLIYIADHSEVKTALLETLDQKIRTAVKEWLHLPPCTCDAILYSSTRDGGLGITKLAGLIPSVQARRLHRIAQSSDDTMKCFMEKEKMEQLHKKLWIQAGGDRENIPSIWEAPPGGMPKRKVSSAEGAAKEEPKRRSARLSAKPPAKVEAKPKKAAAKDKSSDKKVQTKGKRGAKGKQAEVANQETKEDLPAENGETKTEESPASDEAGEKEAKSDGGSSEPPNNVSTNSEWEAPTQKDKFPKPCNWRKNEFKKWTKLASQGRGIVNFERDKISNHWIQYYRRIPHRKLLTALQLRANVYPTREFLARGRQDQYIKACRHCDADIESCAHIIGNCPVTQDARIKRHNYICELLLEEAKKKDWVVFKEPHIRDSNKELYKPDLIFVKDARALVVDVTVRYEAAKSSLEEAAAEKVRKYKHLETEVRHLTNAKDVTFVGFPLGARGKWHQDNFKLLTELGLSKSRQVKMAETFSTVALFSSVDIVHMFASRARKSMVM

SEQ ID NO: 61 - protein, 1783 aa, synthetic construct
SKSWGKFIEEEEAEMASRRNLMIVDGTNLGFRFKHNNSKKPFASSYVSTIQSLAKSYSARTTIVLGDKGKSVFRLEHLPEYKGNRDEKYAQRTEEEKALDEQFFEYLKDAFELCKTTFPTFTIRGVEADDMAAYIVKLIGHLYDHVWLISTDGDWDTLLTDKVSRFSFTTRREYHLRDMYEHHNVDDVEQFISLKAIMGDLGDNIRGVEGIGAKRGYNIIREFGNVLDIIDQLPLPGKQKYIQNLNASEELLFRNLILVDLPTYCVDAIAAVGQDVLDKFTKDILEIAEQASCPKPGPPVSAGAMSLESGLTTHSVLAIERGPNSLANSGSDFGGGGLGLPLRLLRVSVGTQTSRSDWVDLVSWSHPGPTSKSQQVDLVSLFPKHRVDLLSKNDQVDLVAQFLPSKFPPNLAENDLALLVNLEFYRSDLHVYECVHFAAHWEGLSGLPEVYEQLAPQPCVGETLHSSLPRDSELFVPEEGSSEKESEDAPKTSPPTPGKHGLEQTGEEKVMVTVPDKNPPCPCCGTRVNSVLNLIEHLKVSHGKRGVCFRCAKCGKENSNYHSVVCHFPKCRGPETEKAPAGEWICEVCNRDFTTKIGLGQHKRLAHPAVRNQERIVASQPKETSNRGAHKRCWTKEEEELLIRLEAQFEGNKNINKLIAEHITTKTAKQISDKRRLLSRKPAEEPREEPGTCHHTRRAAASLRTEPEMSHHAQAEDRDNGGGMPKRKVSSAEGAAKEEPKRRSARLSAKPPAKVEAKPKKAAAKDKSSDKKVQTKGKRGAKGKQAEVANQETKEDLPAENGETKTEESPASDEAGEKEAKSDGGPGRRPLPGRAAAGGRTMDEIRRHPDKGNGQQRPTKQKSEEQLQAYYKKTLEERLSAGALNTFPRAFKQVMEGRDIKLVINQTAQDCFGCLESISQIRTATRDKKDTVTREKHPKKPFQKWMKDRAIKKGNYLRFQRLFYLDRGKLAKIILDDIECLSCDIPLSEIYSVFKTRWETTGSFKSLGDFKTYGKADNTAFRELITAKEIEKNVQEMSKGSAPGPDGITLGDVVKMDPEFSRTMEIFNLWLTTGKIPDMVRGCRTVLIPKSSKPDRLKDINNWRPITIGSILLRLFSRIVTARLSKACPLNPRQRGFIRAAGCSENLKLLQTIIWSAKREHRPLGVVFVDIAKAFDTVSHQHIIHVLQQREVDPHIVGLVSNMYENISTYITTKRNTHTDKIQIRVGVKQGDPMSPLLFNLAMDPLLCKLEESGKGYHRGQSSITAMAFADDLVLLSDSWENMNTNISILETFCNLTGLKTQGQKCHGFYIKPTKDSYTINDCAAWTINGTPLNMIDPGESEKYLGLRFDPWIGIARSGLSTKLDFWLQRIDQAPLKPLQKTDILKTYTIPRLIYIADHSEVKTALLETLDQKIRTAVKEWLHLPPCTCDAILYSSTRDGGLGITKLAGLIPSVQARRLHRIAQSSDDTMKCFMEKEKMEQLHKKLWIQARGDRENIPSIWEAPPSSEPPNNVSTNSEWEAPTQKDKFPKPCNWRKNEFKKWTKLASQGRGIVNFERDKISNHWIQYYRRIPHRKLLTALQLRANVYPTREFLARGRQDQYIKACRHCDADIESCAHIIGNCPVTQDARIKRHNYICELLLEEAKKKDWVVFKEPHIRDSNKELYKPDLIFVKDARALVVDVTVRYEAAKSSLEEAAAEKVRKYKHLETEVRHLTNAKDVTFVGFPLGARGKWHQDNFKLLTELGLSKSRQVKMAETFSTVALFSSVDIVHMFASRARKSMVM

SEQ ID NO: 62 - protein, 1783 aa, synthetic construct
SKSWGKFIEEEEAEMASRRNLMIVDGTNLGFRFKHNNSKKPFASSYVSTIQSLAKSYSARTTIVLGDKGKSVFRLEHLPEYKGNRDEKYAQRTEEEKALDEQFFEYLKDAFELCKTTFPTFTIRGVEADDMAAYIVKLIGHLYDHVWLISTDGDWDTLLTDKVSRFSFTTRREYHLRDMYEHHNVDDVEQFISLKAIMGDLGDNIRGVEGIGAKRGYNIIREFGNVLDIIDQLPLPGKQKYIQNLNASEELLFRNLILVDLPTYCVDAIAAVGQDVLDKFTKDILEIAEQASCPKPGPPVSAGAMSLESGLTTHSVLAIERGPNSLANSGSDFGGGGLGLPLRLLRVSVGTQTSRSDWVDLVSWSHPGPTSKSQQVDLVSLFPKHRVDLLSKNDQVDLVAQFLPSKFPPNLAENDLALLVNLEFYRSDLHVYECVHFAAHWEGLSGLPEVYEQLAPQPCVGETLHSSLPRDSELFVPEEGSSEKESEDAPKTSPPTPGKHGLEQTGEEKVMVTVPDKNPPCPCCGTRVNSVLNLIEHLKVSHGKRGVCFRCAKCGKENSNYHSVVCHFPKCRGPETEKAPAGEWICEVCNRDFTTKIGLGQHKRLAHPAVRNQERIVASQPKETSNRGAHKRCWTKEEEELLIRLEAQFEGNKNINKLIAEHITTKTAKQISDKRRLLSRKPAEEPREEPGTCHHTRRAAASLRTEPEMSHHAQAEDRDNGGGMPKRKVSSAEGAAKEEPKRRSARLSAKPPAKVEAKPKKAAAKDKSSDKKVQTKGKRGAKGKQAEVANQETKEDLPAENGETKTEESPASDEAGEKEAKSDGGPGRRPLPGRAAAGGRTMDEIRRHPDKGNGQQRPTKQKSEEQLQAYYKKTLEERLSAGALNTFPRAFKQVMEGRDIKLVINQTAQDCFGCLESISQIRTATRDKKDTVTREKHPKKPFQKWMKDRAIKKGNYLRFQRLFYLDRGKLAKIILDDIECLSCDIPLSEIYSVFKTRWETTGSFKSLGDFKTYGKADNTAFRELITAKEIEKNVQEMSKGSAPGPDGITLGDVVKMDPEFSRTMEIFNLWLTTGKIPDMVRGCRTVLIPKSSKPDRLKDINNWRPITIGSILLRLFSRIVTARLSKACPLNPRQRGFIRAAGCSENLKLLQTIIQSAKREHRPLGVVFVDIAKAFDTVSHQHIIHVLQQREVDPHIVGLVSNMYENISTYITTKRNTHTDKIQIRVGVKQGDPMSPLLFNLAMDPLLCKLEESGKGYHRGQSSITAMAFADDLVLLSDSWENMNTNISILETFCNLTGLKTQGQKCHGFYIKPTKDSYTINDCAAWTINGTPLNMIDPGESEKYLGLRFDPWIGIARSGLSTKLDFWLQRIDQAPLKPLQKTDILKTYTIPRLIYIADHSEVKTALLETLDQKIRTAVKEWLHLPPCTCDAILYSSTRDGGLGITKLAGLIPSVQARRLHRIAQSSDDTMKCFMEKEKMEQLHKKLWIQARGDRENIPSIWEAPPSSEPPNNVSTNSEWEAPTQKDKFPKPCNWRKNEFKKWTKLASQGRGIVNFERDKISNHWIQYYRRIPHRKLLTALQLRANVYPTREFLARGRQDQYIKACRHCDADIESCAHIIGNCPVTQDARIKRHNYICELLLEEAKKKDWVVFKEPHIRDSNKELYKPDLIFVKDARALVVDVTVRYEAAKSSLEEAAAEKVRKYKHLETEVRHLTNAKDVTFVGFPLGARGKWHQDNFKLLTELGLSKSRQVKMAETFSTVALFSSVDIVHMFASRARKSMVM

SEQ ID NO: 63 - protein, 1783 aa, synthetic construct
SKSWGKFIEEEEAEMASRRNLMIVDGTNLGFRFKHNNSKKPFASSYVSTIQSLAKSYSARTTIVLGDKGKSVFRLEHLPEYKGNRDEKYAQRTEEEKALDEQFFEYLKDAFELCKTTFPTFTIRGVEADDMAAYIVKLIGHLYDHVWLISTDGDWDTLLTDKVSRFSFTTRREYHLRDMYEHHNVDDVEQFISLKAIMGDLGDNIRGVEGIGAKRGYNIIREFGNVLDIIDQLPLPGKQKYIQNLNASEELLFRNLILVDLPTYCVDAIAAVGQDVLDKFTKDILEIAEQASCPKPGPPVSAGAMSLESGLTTHSVLAIERGPNSLANSGSDFGGGGLGLPLRLLRVSVGTQTSRSDWVDLVSWSHPGPTSKSQQVDLVSLFPKHRVDLLSKNDQVDLVAQFLPSKFPPNLAENDLALLVNLEFYRSDLHVYECVHFAAHWEGLSGLPEVYEQLAPQPCVGETLHSSLPRDSELFVPEEGSSEKESEDAPKTSPPTPGKHGLEQTGEEKVMVTVPDKNPPCPCCGTRVNSVLNLIEHLKVSHGKRGVCFRCAKCGKENSNYHSVVCHFPKCRGPETEKAPAGEWICEVCNRDFTTKIGLGQHKRLAHPAVRNQERIVASQPKETSNRGARKRCWTKEEEELLIRLEAQFEGNKNINKLIAEHITTKTAKQISDKRRLLSRKPAEEPREEPGTCHHTRRAAASLRTEPEMSHHAQAEDRDNGGGMPKRKVSSAEGAAKEEPKRRSARLSAKPPAKVEAKPKKAAAKDKSSDKKVQTKGKRGAKGKQAEVANQETKEDLPAENGETKTEESPASDEAGEKEAKSDGGPGRRPLPGRAAAGGRTMDEIRRHPDKGNGQQRPTKQKSEEQLQAYYKKTLEERLSAGALNTFPRAFKQVMEGRDIKLVINQTAQDCFGCLESISQIRTATRDKKDTVTREKHPKKPFQKWMKDRAIKKGNYLRFQRLFYLDRGKLAKIILDDIECLSCDIPLSEIYSVFKTRWETTGSFKSLGDFKTYGKADNTAFRELITAKEIEKNVQEMSKGSAPGPDGITLGDVVKMDPEFSRTMEIFNLWLTTGKIPDMVRGCRTVLIPKSSKPDRLKDINNWRPITIGSILLRLFSRIVTARLSKACPLNPRQRGFIRAAGCSENLKLLQTIIQSAKREHRPLGVVFVDIAKAFDTVSHQHIIHVLQQREVDPHIVGLVSNMYENISTYITTKRNTHTDKIQIRVGVKQGDPMSPLLFNLAMDPLLCKLEESGKGYHRGQSSITAMAFADDLVLLSDSWENMNTNISILETFCNLTGLKTQGQKCHGFYIKPTKDSYTINDCAAWTINGTPLNMIDPGESEKYLGLRFDPWIGIARSGLSTKLDFWLQRIDQAPLKPLQKTDILKTYTIPRLIYIADHSEVKTALLETLDQKIRTAVKEWLHLPPCTCDAILYSSTRDGGLGITKLAGLIPSVQARRLHRIAQSSDDTMKCFMEKEKMEQLHKKLWIQARGDRENIPSIWEAPPSSEPPNNVSTNSEWEAPTQKDKFPKPCNWRKNEFKKWTKLASQGRGIVNFERDKISNHWIQYYRRIPHRKLLTALQLRANVYPTREFLARGRQDQYIKACRHCDADIESCAHIIGNCPVTQDARIKRHNYICELLLEEAKKKDWVVFKEPHIRDSNKELYKPDLIFVKDARALVVDVTVRYEAAKSSLEEAAAEKVRKYKHLETEVRHLTNAKDVTFVGFPLGARGKWHQDNFKLLTELGLSKSRQVKMAETFSTVALFSSVDIVHMFASRARKSMVM

SEQ ID NO: 64 - protein, 1783 aa, synthetic construct
SKSWGKFIEEEEAEMASRRNLMIVDGTNLGFRFKHNNSKKPFASSYVSTIQSLAKSYSARTTIVLGDKGKSVFRLEHLPEYKGNRDEKYAQRTEEEKALDEQFFEYLKDAFELCKTTFPTFTIRGVEADDMAAYIVKLIGHLYDHVWLISTDGDWDTLLTDKVSRFSFTTRREYHLRDMYEHHNVDDVEQFISLKAIMGDLGDNIRGVEGIGAKRGYNIIREFGNVLDIIDQLPLPGKQKYIQNLNASEELLFRNLILVDLPTYCVDAIAAVGQDVLDKFTKDILEIAEQASCPKPGPPVSAGAMSLESGLTTHSVLAIERGPNSLANSGSDFGGGGLGLPLRLLRVSVGTQTSRSDWVDLVSWSHPGPTSKSQQVDLVSLFPKHRVDLLSKNDQVDLVAQFLPSKFPPNLAENDLALLVNLEFYRSDLHVYECVHFAAHWEGLSGLPEVYEQLAPQPCVGETLHSSLPRDSELFVPEEGSSEKESEDAPKTSPPTPGKHGLEQTGEEKVMVTVPDKNPPCPCCGTRVNSVLNLIEHLKVSHGKRGVCFRCAKCGKENSNYHSVVCHFPKCRGPETEKAPAGEWICEVCNRDFTTKIGLGQHKRLAHPAVRNQERIVASQPKETSNRGARKRCWTKEEEELLIRLEAQFEGNKNINKLIAEHITTKTAKQISDKRRLLSRKPAEEPREEPGTCHHTRRAAASLRTEPEMSHHAQAEDRDNGGGMPKRKVSSAEGAAKEEPKRRSARLSAKPPAKVEAKPKKAAAKDKSSDKKVQTKGKRGAKGKQAEVANQETKEDLPAENGETKTEESPASDEAGEKEAKSDGGPGRRPLPGRAAAGGRTMDEIRRHPDKGNGQQRPTKQKSEEQLQAYYKKTLEERLSAGALNTFPRAFKQVMEGRDIKLVINQTAQDCFGCLESISQIRTATRDKKDTVTREKHPKKPFQKWMKDRAIKKGNYLRFQRLFYLDRGKLAKIILDDIECLSCDIPLSEIYSVFKTRWETTGSFKSLGDFKTYGKADNTAFRELITAKEIEKNVQEMSKGSAPGPDGITLGDVVKMDPEFSRTMEIFNLWLTTGKIPDMVRGCRTVLIPKSSKPDRLKDINNWRPITIGSILLRLFSRIVTARLSKACPLNPRQRGFIRAAGCSENLKLLQTIIWSAKREHRPLGVVFVDIAKAFDTVSHQHIIHVLQQREVDPHIVGLVSNMYENISTYITTKRNTHTDKIQIRVGVKQGDPMSPLLFNLAMDPLLCKLEESGKGYHRGQSSITAMAFADDLVLLSDSWENMNTNISILETFCNLTGLKTQGQKCHGFYIKPTKDSYTINDCAAWTINGTPLNMIDPGESEKYLGLRFDPWIGIARSGLSTKLDFWLQRIDQAPLKPLQKTDILKTYTIPRLIYIADHSEVKTALLETLDQKIRTAVKEWLHLPPCTCDAILYSSTRDGGLGITKLAGLIPSVQARRLHRIAQSSDDTMKCFMEKEKMEQLHKKLWIQARGDRENIPSIWEAPPSSEPPNNVSTNSEWEAPTQKDKFPKPCNWRKNEFKKWTKLASQGRGIVNFERDKISNHWIQYYRRIPHRKLLTALQLRANVYPTREFLARGRQDQYIKACRHCDADIESCAHIIGNCPVTQDARIKRHNYICELLLEEAKKKDWVVFKEPHIRDSNKELYKPDLIFVKDARALVVDVTVRYEAAKSSLEEAAAEKVRKYKHLETEVRHLTNAKDVTFVGFPLGARGKWHQDNFKLLTELGLSKSRQVKMAETFSTVALFSSVDIVHMFASRARKSMVM

SEQ ID NO: 65 - protein, 1878 aa, synthetic construct
SKSWGKFIEEEEAEMASRRNLMIVDGTNLGFRFKHNNSKKPFASSYVSTIQSLAKSYSARTTIVLGDKGKSVFRLEHLPEYKGNRDEKYAQRTEEEKALDEQFFEYLKDAFELCKTTFPTFTIRGVEADDMAAYIVKLIGHLYDHVWLISTDGDWDTLLTDKVSRFSFTTRREYHLRDMYEHHNVDDVEQFISLKAIMGDLGDNIRGVEGIGAKRGYNIIREFGNVLDIIDQLPLPGKQKYIQNLNASEELLFRNLILVDLPTYCVDAIAAVGQDVLDKFTKDILEIAEQASCPKPGPPVSAGAMSLESGLTTHSVLAIERGPNSLANSGSDFGGGGLGLPLRLLRVSVGTQTSRSDWVDLVSWSHPGPTSKSQQVDLVSLFPKHRVDLLSKNDQVDLVAQFLPSKFPPNLAENDLALLVNLEFYRSDLHVYECVHFAAHWEGLSGLPEVYEQLAPQPCVGETLHSSLPRDSELFVPEEGSSEKESEDAPKTSPPTPGKHGLEQTGEEKVMVTVPDKNPPCPCCGTRVNSVLNLIEHLKVSHGKRGVCFRCAKCGKENSNYHSVVCHFPKCRGPETEKAPAGEWICEVCNRDFTTKIGLGQHKRLAHPAVRNQERIVASQPKETSNRGAHKRCWTKEEEELLIRLEAQFEGNKNINKLIAEHITTKTAKQISDKRRLLSRKPAEEPREEPGTCHHTRRAAASLRTEPEMSHHAQAEDRDNGGGDILAEAHGTRPDLTDQPLPDADHTWYTDGSSLLQEGQRKAGAAVTTETEVIWAKALPAGTSAQRAELIALTQALKMAEGKKLNVYTDSRYAFATAHIHGEIYRRRGWLTSEGKEIKNKDEILALLKALFLPKRLSIIHCPGHQKGHSAEARGNRMADQAARKAAITETPDTSTLLIENSSPSGGSKRTADGSEFEGGPGRRPLPGRAAAGGRTMDEIRRHPDKGNGQQRPTKQKSEEQLQAYYKKTLEERLSAGALNTFPRAFKQVMEGRDIKLVINQTAQDCFGCLESISQIRTATRDKKDTVTREKHPKKPFQKWMKDRAIKKGNYLRFQRLFYLDRGKLAKIILDDIECLSCDIPLSEIYSVFKTRWETTGSFKSLGDFKTYGKADNTAFRELITAKEIEKNVQEMSKGSAPGPDGITLGDVVKMDPEFSRTMEIFNLWLTTGKIPDMVRGCRTVLIPKSSKPDRLKDINNWRPITIGSILLRLFSRIVTARLSKACPLNPRQRGFIRAAGCSENLKLLQTIIWSAKREHRPLGVVFVDIAKAFDTVSHQHIIHVLQQREVDPHIVGLVSNMYENISTYITTKRNTHTDKIQIRVGVKQGDPMSPLLFNLAMDPLLCKLEESGKGYHRGQSSITAMAFADDLVLLSDSWENMNTNISILETFCNLTGLKTQGQKCHGFYIKPTKDSYTINDCAAWTINGTPLNMIDPGESEKYLGLRFDPWIGIARSGLSTKLDFWLQRIDQAPLKPLQKTDILKTYTIPRLIYIADHSEVKTALLETLDQKIRTAVKEWLHLPPCTCDAILYSSTRDGGLGITKLAGLIPSVQARRLHRIAQSSDDTMKCFMEKEKMEQLHKKLWIQARGDRENIPSIWEAPPSSEPPNNVSTNSEWEAPTQKDKFPKPCNWRKNEFKKWTKLASQGRGIVNFERDKISNHWIQYYRRIPHRKLLTALQLRANVYPTREFLARGRQDQYIKACRHCDADIESCAHIIGNCPVTQDARIKRHNYICELLLEEAKKKDWVVFKEPHIRDSNKELYKPDLIFVKDARALVVDVTVRYEAAKSSLEEAAAEKVRKYKHLETEVRHLTNAKDVTFVGFPLGARGKWHQDNFKLLTELGLSKSRQVKMAETFSTVALFSSVDIVHMFASRARKSMVM

SEQ ID NO: 66 - protein, 1878 aa, synthetic construct
SKSWGKFIEEEEAEMASRRNLMIVDGTNLGFRFKHNNSKKPFASSYVSTIQSLAKSYSARTTIVLGDKGKSVFRLEHLPEYKGNRDEKYAQRTEEEKALDEQFFEYLKDAFELCKTTFPTFTIRGVEADDMAAYIVKLIGHLYDHVWLISTDGDWDTLLTDKVSRFSFTTRREYHLRDMYEHHNVDDVEQFISLKAIMGDLGDNIRGVEGIGAKRGYNIIREFGNVLDIIDQLPLPGKQKYIQNLNASEELLFRNLILVDLPTYCVDAIAAVGQDVLDKFTKDILEIAEQASCPKPGPPVSAGAMSLESGLTTHSVLAIERGPNSLANSGSDFGGGGLGLPLRLLRVSVGTQTSRSDWVDLVSWSHPGPTSKSQQVDLVSLFPKHRVDLLSKNDQVDLVAQFLPSKFPPNLAENDLALLVNLEFYRSDLHVYECVHFAAHWEGLSGLPEVYEQLAPQPCVGETLHSSLPRDSELFVPEEGSSEKESEDAPKTSPPTPGKHGLEQTGEEKVMVTVPDKNPPCPCCGTRVNSVLNLIEHLKVSHGKRGVCFRCAKCGKENSNYHSVVCHFPKCRGPETEKAPAGEWICEVCNRDFTTKIGLGQHKRLAHPAVRNQERIVASQPKETSNRGAHKRCWTKEEEELLIRLEAQFEGNKNINKLIAEHITTKTAKQISDKRRLLSRKPAEEPREEPGTCHHTRRAAASLRTEPEMSHHAQAEDRDNGGGDILAEAHGTRPDLTDQPLPDADHTWYTDGSSLLQEGQRKAGAAVTTETEVIWAKALPAGTSAQRAELIALTQALKMAEGKKLNVYTDSRYAFATAHIHGEIYRRRGWLTSEGKEIKNKDEILALLKALFLPKRLSIIHCPGHQKGHSAEARGNRMADQAARKAAITETPDTSTLLIENSSPSGGSKRTADGSEFEGGPGRRPLPGRAAAGGRTMDEIRRHPDKGNGQQRPTKQKSEEQLQAYYKKTLEERLSAGALNTFPRAFKQVMEGRDIKLVINQTAQDCFGCLESISQIRTATRDKKDTVTREKHPKKPFQKWMKDRAIKKGNYLRFQRLFYLDRGKLAKIILDDIECLSCDIPLSEIYSVFKTRWETTGSFKSLGDFKTYGKADNTAFRELITAKEIEKNVQEMSKGSAPGPDGITLGDVVKMDPEFSRTMEIFNLWLTTGKIPDMVRGCRTVLIPKSSKPDRLKDINNWRPITIGSILLRLFSRIVTARLSKACPLNPRQRGFIRAAGCSENLKLLQTIIQSAKREHRPLGVVFVDIAKAFDTVSHQHIIHVLQQREVDPHIVGLVSNMYENISTYITTKRNTHTDKIQIRVGVKQGDPMSPLLFNLAMDPLLCKLEESGKGYHRGQSSITAMAFADDLVLLSDSWENMNTNISILETFCNLTGLKTQGQKCHGFYIKPTKDSYTINDCAAWTINGTPLNMIDPGESEKYLGLRFDPWIGIARSGLSTKLDFWLQRIDQAPLKPLQKTDILKTYTIPRLIYIADHSEVKTALLETLDQKIRTAVKEWLHLPPCTCDAILYSSTRDGGLGITKLAGLIPSVQARRLHRIAQSSDDTMKCFMEKEKMEQLHKKLWIQARGDRENIPSIWEAPPSSEPPNNVSTNSEWEAPTQKDKFPKPCNWRKNEFKKWTKLASQGRGIVNFERDKISNHWIQYYRRIPHRKLLTALQLRANVYPTREFLARGRQDQYIKACRHCDADIESCAHIIGNCPVTQDARIKRHNYICELLLEEAKKKDWVVFKEPHIRDSNKELYKPDLIFVKDARALVVDVTVRYEAAKSSLEEAAAEKVRKYKHLETEVRHLTNAKDVTFVGFPLGARGKWHQDNFKLLTELGLSKSRQVKMAETFSTVALFSSVDIVHMFASRARKSMVM

SEQ ID NO: 67 - protein, 1878 aa, synthetic construct
SKSWGKFIEEEEAEMASRRNLMIVDGTNLGFRFKHNNSKKPFASSYVSTIQSLAKSYSARTTIVLGDKGKSVFRLEHLPEYKGNRDEKYAQRTEEEKALDEQFFEYLKDAFELCKTTFPTFTIRGVEADDMAAYIVKLIGHLYDHVWLISTDGDWDTLLTDKVSRFSFTTRREYHLRDMYEHHNVDDVEQFISLKAIMGDLGDNIRGVEGIGAKRGYNIIREFGNVLDIIDQLPLPGKQKYIQNLNASEELLFRNLILVDLPTYCVDAIAAVGQDVLDKFTKDILEIAEQASCPKPGPPVSAGAMSLESGLTTHSVLAIERGPNSLANSGSDFGGGGLGLPLRLLRVSVGTQTSRSDWVDLVSWSHPGPTSKSQQVDLVSLFPKHRVDLLSKNDQVDLVAQFLPSKFPPNLAENDLALLVNLEFYRSDLHVYECVHFAAHWEGLSGLPEVYEQLAPQPCVGETLHSSLPRDSELFVPEEGSSEKESEDAPKTSPPTPGKHGLEQTGEEKVMVTVPDKNPPCPCCGTRVNSVLNLIEHLKVSHGKRGVCFRCAKCGKENSNYHSVVCHFPKCRGPETEKAPAGEWICEVCNRDFTTKIGLGQHKRLAHPAVRNQERIVASQPKETSNRGARKRCWTKEEEELLIRLEAQFEGNKNINKLIAEHITTKTAKQISDKRRLLSRKPAEEPREEPGTCHHTRRAAASLRTEPEMSHHAQAEDRDNGGGDILAEAHGTRPDLTDQPLPDADHTWYTDGSSLLQEGQRKAGAAVTTETEVIWAKALPAGTSAQRAELIALTQALKMAEGKKLNVYTDSRYAFATAHIHGEIYRRRGWLTSEGKEIKNKDEILALLKALFLPKRLSIIHCPGHQKGHSAEARGNRMADQAARKAAITETPDTSTLLIENSSPSGGSKRTADGSEFEGGPGRRPLPGRAAAGGRTMDEIRRHPDKGNGQQRPTKQKSEEQLQAYYKKTLEERLSAGALNTFPRAFKQVMEGRDIKLVINQTAQDCFGCLESISQIRTATRDKKDTVTREKHPKKPFQKWMKDRAIKKGNYLRFQRLFYLDRGKLAKIILDDIECLSCDIPLSEIYSVFKTRWETTGSFKSLGDFKTYGKADNTAFRELITAKEIEKNVQEMSKGSAPGPDGITLGDVVKMDPEFSRTMEIFNLWLTTGKIPDMVRGCRTVLIPKSSKPDRLKDINNWRPITIGSILLRLFSRIVTARLSKACPLNPRQRGFIRAAGCSENLKLLQTIIQSAKREHRPLGVVFVDIAKAFDTVSHQHIIHVLQQREVDPHIVGLVSNMYENISTYITTKRNTHTDKIQIRVGVKQGDPMSPLLFNLAMDPLLCKLEESGKGYHRGQSSITAMAFADDLVLLSDSWENMNTNISILETFCNLTGLKTQGQKCHGFYIKPTKDSYTINDCAAWTINGTPLNMIDPGESEKYLGLRFDPWIGIARSGLSTKLDFWLQRIDQAPLKPLQKTDILKTYTIPRLIYIADHSEVKTALLETLDQKIRTAVKEWLHLPPCTCDAILYSSTRDGGLGITKLAGLIPSVQARRLHRIAQSSDDTMKCFMEKEKMEQLHKKLWIQARGDRENIPSIWEAPPSSEPPNNVSTNSEWEAPTQKDKFPKPCNWRKNEFKKWTKLASQGRGIVNFERDKISNHWIQYYRRIPHRKLLTALQLRANVYPTREFLARGRQDQYIKACRHCDADIESCAHIIGNCPVTQDARIKRHNYICELLLEEAKKKDWVVFKEPHIRDSNKELYKPDLIFVKDARALVVDVTVRYEAAKSSLEEAAAEKVRKYKHLETEVRHLTNAKDVTFVGFPLGARGKWHQDNFKLLTELGLSKSRQVKMAETFSTVALFSSVDIVHMFASRARKSMVM

SEQ ID NO: 68 - protein, 1878 aa, synthetic construct
SKSWGKFIEEEEAEMASRRNLMIVDGTNLGFRFKHNNSKKPFASSYVSTIQSLAKSYSARTTIVLGDKGKSVFRLEHLPEYKGNRDEKYAQRTEEEKALDEQFFEYLKDAFELCKTTFPTFTIRGVEADDMAAYIVKLIGHLYDHVWLISTDGDWDTLLTDKVSRFSFTTRREYHLRDMYEHHNVDDVEQFISLKAIMGDLGDNIRGVEGIGAKRGYNIIREFGNVLDIIDQLPLPGKQKYIQNLNASEELLFRNLILVDLPTYCVDAIAAVGQDVLDKFTKDILEIAEQASCPKPGPPVSAGAMSLESGLTTHSVLAIERGPNSLANSGSDFGGGGLGLPLRLLRVSVGTQTSRSDWVDLVSWSHPGPTSKSQQVDLVSLFPKHRVDLLSKNDQVDLVAQFLPSKFPPNLAENDLALLVNLEFYRSDLHVYECVHFAAHWEGLSGLPEVYEQLAPQPCVGETLHSSLPRDSELFVPEEGSSEKESEDAPKTSPPTPGKHGLEQTGEEKVMVTVPDKNPPCPCCGTRVNSVLNLIEHLKVSHGKRGVCFRCAKCGKENSNYHSVVCHFPKCRGPETEKAPAGEWICEVCNRDFTTKIGLGQHKRLAHPAVRNQERIVASQPKETSNRGARKRCWTKEEEELLIRLEAQFEGNKNINKLIAEHITTKTAKQISDKRRLLSRKPAEEPREEPGTCHHTRRAAASLRTEPEMSHHAQAEDRDNGGGDILAEAHGTRPDLTDQPLPDADHTWYTDGSSLLQEGQRKAGAAVTTETEVIWAKALPAGTSAQRAELIALTQALKMAEGKKLNVYTDSRYAFATAHIHGEIYRRRGWLTSEGKEIKNKDEILALLKALFLPKRLSIIHCPGHQKGHSAEARGNRMADQAARKAAITETPDTSTLLIENSSPSGGSKRTADGSEFEGGPGRRPLPGRAAAGGRTMDEIRRHPDKGNGQQRPTKQKSEEQLQAYYKKTLEERLSAGALNTFPRAFKQVMEGRDIKLVINQTAQDCFGCLESISQIRTATRDKKDTVTREKHPKKPFQKWMKDRAIKKGNYLRFQRLFYLDRGKLAKIILDDIECLSCDIPLSEIYSVFKTRWETTGSFKSLGDFKTYGKADNTAFRELITAKEIEKNVQEMSKGSAPGPDGITLGDVVKMDPEFSRTMEIFNLWLTTGKIPDMVRGCRTVLIPKSSKPDRLKDINNWRPITIGSILLRLFSRIVTARLSKACPLNPRQRGFIRAAGCSENLKLLQTIIWSAKREHRPLGVVFVDIAKAFDTVSHQHIIHVLQQREVDPHIVGLVSNMYENISTYITTKRNTHTDKIQIRVGVKQGDPMSPLLFNLAMDPLLCKLEESGKGYHRGQSSITAMAFADDLVLLSDSWENMNTNISILETFCNLTGLKTQGQKCHGFYIKPTKDSYTINDCAAWTINGTPLNMIDPGESEKYLGLRFDPWIGIARSGLSTKLDFWLQRIDQAPLKPLQKTDILKTYTIPRLIYIADHSEVKTALLETLDQKIRTAVKEWLHLPPCTCDAILYSSTRDGGLGITKLAGLIPSVQARRLHRIAQSSDDTMKCFMEKEKMEQLHKKLWIQARGDRENIPSIWEAPPSSEPPNNVSTNSEWEAPTQKDKFPKPCNWRKNEFKKWTKLASQGRGIVNFERDKISNHWIQYYRRIPHRKLLTALQLRANVYPTREFLARGRQDQYIKACRHCDADIESCAHIIGNCPVTQDARIKRHNYICELLLEEAKKKDWVVFKEPHIRDSNKELYKPDLIFVKDARALVVDVTVRYEAAKSSLEEAAAEKVRKYKHLETEVRHLTNAKDVTFVGFPLGARGKWHQDNFKLLTELGLSKSRQVKMAETFSTVALFSSVDIVHMFASRARKSMVM

SEQ ID NO: 69 - protein, 1556 aa, synthetic construct
VTVKFKYKGEELEVDISKIKKVWRVGKMISFTYDDNGKTGRGAVSEKDAPKELLQMLEKSGKKASCPKPGPPVSAGAMSLESGLTTHSVLAIERGPNSLANSGSDFGGGGLGLPLRLLRVSVGTQTSRSDWVDLVSWSHPGPTSKSQQVDLVSLFPKHRVDLLSKNDQVDLVAQFLPSKFPPNLAENDLALLVNLEFYRSDLHVYECVHFAAHWEGLSGLPEVYEQLAPQPCVGETLHSSLPRDSELFVPEEGSSEKESEDAPKTSPPTPGKHGLEQTGEEKVMVTVPDKNPPCPCCGTRVNSVLNLIEHLKVSHGKRGVCFRCAKCGKENSNYHSVVCHFPKCRGPETEKAPAGEWICEVCNRDFTTKIGLGQHKRLAHPAVRNQERIVASQPKETSNRGAHKRCWTKEEEELLIRLEAQFEGNKNINKLIAEHITTKTAKQISDKRRLLSRKPAEEPREEPGTCHHTRRAAASLRTEPEMSHHAQAEDRDNGGGMPKRKVSSAEGAAKEEPKRRSARLSAKPPAKVEAKPKKAAAKDKSSDKKVQTKGKRGAKGKQAEVANQETKEDLPAENGETKTEESPASDEAGEKEAKSDGGPGRRPLPGRAAAGGRTMDEIRRHPDKGNGQQRPTKQKSEEQLQAYYKKTLEERLSAGALNTFPRAFKQVMEGRDIKLVINQTAQDCFGCLESISQIRTATRDKKDTVTREKHPKKPFQKWMKDRAIKKGNYLRFQRLFYLDRGKLAKIILDDIECLSCDIPLSEIYSVFKTRWETTGSFKSLGDFKTYGKADNTAFRELITAKEIEKNVQEMSKGSAPGPDGITLGDVVKMDPEFSRTMEIFNLWLTTGKIPDMVRGCRTVLIPKSSKPDRLKDINNWRPITIGSILLRLFSRIVTARLSKACPLNPRQRGFIRAAGCSENLKLLQTIIWSAKREHRPLGVVFVDIAKAFDTVSHQHIIHVLQQREVDPHIVGLVSNMYENISTYITTKRNTHTDKIQIRVGVKQGDPMSPLLFNLAMDPLLCKLEESGKGYHRGQSSITAMAFADDLVLLSDSWENMNTNISILETFCNLTGLKTQGQKCHGFYIKPTKDSYTINDCAAWTINGTPLNMIDPGESEKYLGLRFDPWIGIARSGLSTKLDFWLQRIDQAPLKPLQKTDILKTYTIPRLIYIADHSEVKTALLETLDQKIRTAVKEWLHLPPCTCDAILYSSTRDGGLGITKLAGLIPSVQARRLHRIAQSSDDTMKCFMEKEKMEQLHKKLWIQARGDRENIPSIWEAPPSSEPPNNVSTNSEWEAPTQKDKFPKPCNWRKNEFKKWTKLASQGRGIVNFERDKISNHWIQYYRRIPHRKLLTALQLRANVYPTREFLARGRQDQYIKACRHCDADIESCAHIIGNCPVTQDARIKRHNYICELLLEEAKKKDWVVFKEPHIRDSNKELYKPDLIFVKDARALVVDVTVRYEAAKSSLEEAAAEKVRKYKHLETEVRHLTNAKDVTFVGFPLGARGKWHQDNFKLLTELGLSKSRQVKMAETFSTVALFSSVDIVHMFASRARKSMVM

SEQ ID NO: 70 - protein, 1556 aa, synthetic construct
VTVKFKYKGEELEVDISKIKKVWRVGKMISFTYDDNGKTGRGAVSEKDAPKELLQMLEKSGKKASCPKPGPPVSAGAMSLESGLTTHSVLAIERGPNSLANSGSDFGGGGLGLPLRLLRVSVGTQTSRSDWVDLVSWSHPGPTSKSQQVDLVSLFPKHRVDLLSKNDQVDLVAQFLPSKFPPNLAENDLALLVNLEFYRSDLHVYECVHFAAHWEGLSGLPEVYEQLAPQPCVGETLHSSLPRDSELFVPEEGSSEKESEDAPKTSPPTPGKHGLEQTGEEKVMVTVPDKNPPCPCCGTRVNSVLNLIEHLKVSHGKRGVCFRCAKCGKENSNYHSVVCHFPKCRGPETEKAPAGEWICEVCNRDFTTKIGLGQHKRLAHPAVRNQERIVASQPKETSNRGAHKRCWTKEEEELLIRLEAQFEGNKNINKLIAEHITTKTAKQISDKRRLLSRKPAEEPREEPGTCHHTRRAAASLRTEPEMSHHAQAEDRDNGGGMPKRKVSSAEGAAKEEPKRRSARLSAKPPAKVEAKPKKAAAKDKSSDKKVQTKGKRGAKGKQAEVANQETKEDLPAENGETKTEESPASDEAGEKEAKSDGGPGRRPLPGRAAAGGRTMDEIRRHPDKGNGQQRPTKQKSEEQLQAYYKKTLEERLSAGALNTFPRAFKQVMEGRDIKLVINQTAQDCFGCLESISQIRTATRDKKDTVTREKHPKKPFQKWMKDRAIKKGNYLRFQRLFYLDRGKLAKIILDDIECLSCDIPLSEIYSVFKTRWETTGSFKSLGDFKTYGKADNTAFRELITAKEIEKNVQEMSKGSAPGPDGITLGDVVKMDPEFSRTMEIFNLWLTTGKIPDMVRGCRTVLIPKSSKPDRLKDINNWRPITIGSILLRLFSRIVTARLSKACPLNPRQRGFIRAAGCSENLKLLQTIIQSAKREHRPLGVVFVDIAKAFDTVSHQHIIHVLQQREVDPHIVGLVSNMYENISTYITTKRNTHTDKIQIRVGVKQGDPMSPLLFNLAMDPLLCKLEESGKGYHRGQSSITAMAFADDLVLLSDSWENMNTNISILETFCNLTGLKTQGQKCHGFYIKPTKDSYTINDCAAWTINGTPLNMIDPGESEKYLGLRFDPWIGIARSGLSTKLDFWLQRIDQAPLKPLQKTDILKTYTIPRLIYIADHSEVKTALLETLDQKIRTAVKEWLHLPPCTCDAILYSSTRDGGLGITKLAGLIPSVQARRLHRIAQSSDDTMKCFMEKEKMEQLHKKLWIQARGDRENIPSIWEAPPSSEPPNNVSTNSEWEAPTQKDKFPKPCNWRKNEFKKWTKLASQGRGIVNFERDKISNHWIQYYRRIPHRKLLTALQLRANVYPTREFLARGRQDQYIKACRHCDADIESCAHIIGNCPVTQDARIKRHNYICELLLEEAKKKDWVVFKEPHIRDSNKELYKPDLIFVKDARALVVDVTVRYEAAKSSLEEAAAEKVRKYKHLETEVRHLTNAKDVTFVGFPLGARGKWHQDNFKLLTELGLSKSRQVKMAETFSTVALFSSVDIVHMFASRARKSMVM

SEQ ID NO: 71 - protein, 1556 aa, synthetic construct
VTVKFKYKGEELEVDISKIKKVWRVGKMISFTYDDNGKTGRGAVSEKDAPKELLQMLEKSGKKASCPKPGPPVSAGAMSLESGLTTHSVLAIERGPNSLANSGSDFGGGGLGLPLRLLRVSVGTQTSRSDWVDLVSWSHPGPTSKSQQVDLVSLFPKHRVDLLSKNDQVDLVAQFLPSKFPPNLAENDLALLVNLEFYRSDLHVYECVHFAAHWEGLSGLPEVYEQLAPQPCVGETLHSSLPRDSELFVPEEGSSEKESEDAPKTSPPTPGKHGLEQTGEEKVMVTVPDKNPPCPCCGTRVNSVLNLIEHLKVSHGKRGVCFRCAKCGKENSNYHSVVCHFPKCRGPETEKAPAGEWICEVCNRDFTTKIGLGQHKRLAHPAVRNQERIVASQPKETSNRGARKRCWTKEEEELLIRLEAQFEGNKNINKLIAEHITTKTAKQISDKRRLLSRKPAEEPREEPGTCHHTRRAAASLRTEPEMSHHAQAEDRDNGGGMPKRKVSSAEGAAKEEPKRRSARLSAKPPAKVEAKPKKAAAKDKSSDKKVQTKGKRGAKGKQAEVANQETKEDLPAENGETKTEESPASDEAGEKEAKSDGGPGRRPLPGRAAAGGRTMDEIRRHPDKGNGQQRPTKQKSEEQLQAYYKKTLEERLSAGALNTFPRAFKQVMEGRDIKLVINQTAQDCFGCLESISQIRTATRDKKDTVTREKHPKKPFQKWMKDRAIKKGNYLRFQRLFYLDRGKLAKIILDDIECLSCDIPLSEIYSVFKTRWETTGSFKSLGDFKTYGKADNTAFRELITAKEIEKNVQEMSKGSAPGPDGITLGDVVKMDPEFSRTMEIFNLWLTTGKIPDMVRGCRTVLIPKSSKPDRLKDINNWRPITIGSILLRLFSRIVTARLSKACPLNPRQRGFIRAAGCSENLKLLQTIIQSAKREHRPLGVVFVDIAKAFDTVSHQHIIHVLQQREVDPHIVGLVSNMYENISTYITTKRNTHTDKIQIRVGVKQGDPMSPLLFNLAMDPLLCKLEESGKGYHRGQSSITAMAFADDLVLLSDSWENMNTNISILETFCNLTGLKTQGQKCHGFYIKPTKDSYTINDCAAWTINGTPLNMIDPGESEKYLGLRFDPWIGIARSGLSTKLDFWLQRIDQAPLKPLQKTDILKTYTIPRLIYIADHSEVKTALLETLDQKIRTAVKEWLHLPPCTCDAILYSSTRDGGLGITKLAGLIPSVQARRLHRIAQSSDDTMKCFMEKEKMEQLHKKLWIQARGDRENIPSIWEAPPSSEPPNNVSTNSEWEAPTQKDKFPKPCNWRKNEFKKWTKLASQGRGIVNFERDKISNHWIQYYRRIPHRKLLTALQLRANVYPTREFLARGRQDQYIKACRHCDADIESCAHIIGNCPVTQDARIKRHNYICELLLEEAKKKDWVVFKEPHIRDSNKELYKPDLIFVKDARALVVDVTVRYEAAKSSLEEAAAEKVRKYKHLETEVRHLTNAKDVTFVGFPLGARGKWHQDNFKLLTELGLSKSRQVKMAETFSTVALFSSVDIVHMFASRARKSMVM

SEQ ID NO: 72 - protein, 1556 aa, synthetic construct
VTVKFKYKGEELEVDISKIKKVWRVGKMISFTYDDNGKTGRGAVSEKDAPKELLQMLEKSGKKASCPKPGPPVSAGAMSLESGLTTHSVLAIERGPNSLANSGSDFGGGGLGLPLRLLRVSVGTQTSRSDWVDLVSWSHPGPTSKSQQVDLVSLFPKHRVDLLSKNDQVDLVAQFLPSKFPPNLAENDLALLVNLEFYRSDLHVYECVHFAAHWEGLSGLPEVYEQLAPQPCVGETLHSSLPRDSELFVPEEGSSEKESEDAPKTSPPTPGKHGLEQTGEEKVMVTVPDKNPPCPCCGTRVNSVLNLIEHLKVSHGKRGVCFRCAKCGKENSNYHSVVCHFPKCRGPETEKAPAGEWICEVCNRDFTTKIGLGQHKRLAHPAVRNQERIVASQPKETSNRGARKRCWTKEEEELLIRLEAQFEGNKNINKLIAEHITTKTAKQISDKRRLLSRKPAEEPREEPGTCHHTRRAAASLRTEPEMSHHAQAEDRDNGGGMPKRKVSSAEGAAKEEPKRRSARLSAKPPAKVEAKPKKAAAKDKSSDKKVQTKGKRGAKGKQAEVANQETKEDLPAENGETKTEESPASDEAGEKEAKSDGGPGRRPLPGRAAAGGRTMDEIRRHPDKGNGQQRPTKQKSEEQLQAYYKKTLEERLSAGALNTFPRAFKQVMEGRDIKLVINQTAQDCFGCLESISQIRTATRDKKDTVTREKHPKKPFQKWMKDRAIKKGNYLRFQRLFYLDRGKLAKIILDDIECLSCDIPLSEIYSVFKTRWETTGSFKSLGDFKTYGKADNTAFRELITAKEIEKNVQEMSKGSAPGPDGITLGDVVKMDPEFSRTMEIFNLWLTTGKIPDMVRGCRTVLIPKSSKPDRLKDINNWRPITIGSILLRLFSRIVTARLSKACPLNPRQRGFIRAAGCSENLKLLQTIIWSAKREHRPLGVVFVDIAKAFDTVSHQHIIHVLQQREVDPHIVGLVSNMYENISTYITTKRNTHTDKIQIRVGVKQGDPMSPLLFNLAMDPLLCKLEESGKGYHRGQSSITAMAFADDLVLLSDSWENMNTNISILETFCNLTGLKTQGQKCHGFYIKPTKDSYTINDCAAWTINGTPLNMIDPGESEKYLGLRFDPWIGIARSGLSTKLDFWLQRIDQAPLKPLQKTDILKTYTIPRLIYIADHSEVKTALLETLDQKIRTAVKEWLHLPPCTCDAILYSSTRDGGLGITKLAGLIPSVQARRLHRIAQSSDDTMKCFMEKEKMEQLHKKLWIQARGDRENIPSIWEAPPSSEPPNNVSTNSEWEAPTQKDKFPKPCNWRKNEFKKWTKLASQGRGIVNFERDKISNHWIQYYRRIPHRKLLTALQLRANVYPTREFLARGRQDQYIKACRHCDADIESCAHIIGNCPVTQDARIKRHNYICELLLEEAKKKDWVVFKEPHIRDSNKELYKPDLIFVKDARALVVDVTVRYEAAKSSLEEAAAEKVRKYKHLETEVRHLTNAKDVTFVGFPLGARGKWHQDNFKLLTELGLSKSRQVKMAETFSTVALFSSVDIVHMFASRARKSMVM

SEQ ID NO: 73 - protein, 1651 aa, synthetic construct
VTVKFKYKGEELEVDISKIKKVWRVGKMISFTYDDNGKTGRGAVSEKDAPKELLQMLEKSGKKASCPKPGPPVSAGAMSLESGLTTHSVLAIERGPNSLANSGSDFGGGGLGLPLRLLRVSVGTQTSRSDWVDLVSWSHPGPTSKSQQVDLVSLFPKHRVDLLSKNDQVDLVAQFLPSKFPPNLAENDLALLVNLEFYRSDLHVYECVHFAAHWEGLSGLPEVYEQLAPQPCVGETLHSSLPRDSELFVPEEGSSEKESEDAPKTSPPTPGKHGLEQTGEEKVMVTVPDKNPPCPCCGTRVNSVLNLIEHLKVSHGKRGVCFRCAKCGKENSNYHSVVCHFPKCRGPETEKAPAGEWICEVCNRDFTTKIGLGQHKRLAHPAVRNQERIVASQPKETSNRGAHKRCWTKEEEELLIRLEAQFEGNKNINKLIAEHITTKTAKQISDKRRLLSRKPAEEPREEPGTCHHTRRAAASLRTEPEMSHHAQAEDRDNGGGDILAEAHGTRPDLTDQPLPDADHTWYTDGSSLLQEGQRKAGAAVTTETEVIWAKALPAGTSAQRAELIALTQALKMAEGKKLNVYTDSRYAFATAHIHGEIYRRRGWLTSEGKEIKNKDEILALLKALFLPKRLSIIHCPGHQKGHSAEARGNRMADQAARKAAITETPDTSTLLIENSSPSGGSKRTADGSEFEGGPGRRPLPGRAAAGGRTMDEIRRHPDKGNGQQRPTKQKSEEQLQAYYKKTLEERLSAGALNTFPRAFKQVMEGRDIKLVINQTAQDCFGCLESISQIRTATRDKKDTVTREKHPKKPFQKWMKDRAIKKGNYLRFQRLFYLDRGKLAKIILDDIECLSCDIPLSEIYSVFKTRWETTGSFKSLGDFKTYGKADNTAFRELITAKEIEKNVQEMSKGSAPGPDGITLGDVVKMDPEFSRTMEIFNLWLTTGKIPDMVRGCRTVLIPKSSKPDRLKDINNWRPITIGSILLRLFSRIVTARLSKACPLNPRQRGFIRAAGCSENLKLLQTIIWSAKREHRPLGVVFVDIAKAFDTVSHQHIIHVLQQREVDPHIVGLVSNMYENISTYITTKRNTHTDKIQIRVGVKQGDPMSPLLFNLAMDPLLCKLEESGKGYHRGQSSITAMAFADDLVLLSDSWENMNTNISILETFCNLTGLKTQGQKCHGFYIKPTKDSYTINDCAAWTINGTPLNMIDPGESEKYLGLRFDPWIGIARSGLSTKLDFWLQRIDQAPLKPLQKTDILKTYTIPRLIYIADHSEVKTALLETLDQKIRTAVKEWLHLPPCTCDAILYSSTRDGGLGITKLAGLIPSVQARRLHRIAQSSDDTMKCFMEKEKMEQLHKKLWIQARGDRENIPSIWEAPPSSEPPNNVSTNSEWEAPTQKDKFPKPCNWRKNEFKKWTKLASQGRGIVNFERDKISNHWIQYYRRIPHRKLLTALQLRANVYPTREFLARGRQDQYIKACRHCDADIESCAHIIGNCPVTQDARIKRHNYICELLLEEAKKKDWVVFKEPHIRDSNKELYKPDLIFVKDARALVVDVTVRYEAAKSSLEEAAAEKVRKYKHLETEVRHLTNAKDVTFVGFPLGARGKWHQDNFKLLTELGLSKSRQVKMAETFSTVALFSSVDIVHMFASRARKSMVM

SEQ ID NO: 74 - protein, 1651 aa, synthetic construct
VTVKFKYKGEELEVDISKIKKVWRVGKMISFTYDDNGKTGRGAVSEKDAPKELLQMLEKSGKKASCPKPGPPVSAGAMSLESGLTTHSVLAIERGPNSLANSGSDFGGGGLGLPLRLLRVSVGTQTSRSDWVDLVSWSHPGPTSKSQQVDLVSLFPKHRVDLLSKNDQVDLVAQFLPSKFPPNLAENDLALLVNLEFYRSDLHVYECVHFAAHWEGLSGLPEVYEQLAPQPCVGETLHSSLPRDSELFVPEEGSSEKESEDAPKTSPPTPGKHGLEQTGEEKVMVTVPDKNPPCPCCGTRVNSVLNLIEHLKVSHGKRGVCFRCAKCGKENSNYHSVVCHFPKCRGPETEKAPAGEWICEVCNRDFTTKIGLGQHKRLAHPAVRNQERIVASQPKETSNRGAHKRCWTKEEEELLIRLEAQFEGNKNINKLIAEHITTKTAKQISDKRRLLSRKPAEEPREEPGTCHHTRRAAASLRTEPEMSHHAQAEDRDNGGGDILAEAHGTRPDLTDQPLPDADHTWYTDGSSLLQEGQRKAGAAVTTETEVIWAKALPAGTSAQRAELIALTQALKMAEGKKLNVYTDSRYAFATAHIHGEIYRRRGWLTSEGKEIKNKDEILALLKALFLPKRLSIIHCPGHQKGHSAEARGNRMADQAARKAAITETPDTSTLLIENSSPSGGSKRTADGSEFEGGPGRRPLPGRAAAGGRTMDEIRRHPDKGNGQQRPTKQKSEEQLQAYYKKTLEERLSAGALNTFPRAFKQVMEGRDIKLVINQTAQDCFGCLESISQIRTATRDKKDTVTREKHPKKPFQKWMKDRAIKKGNYLRFQRLFYLDRGKLAKIILDDIECLSCDIPLSEIYSVFKTRWETTGSFKSLGDFKTYGKADNTAFRELITAKEIEKNVQEMSKGSAPGPDGITLGDVVKMDPEFSRTMEIFNLWLTTGKIPDMVRGCRTVLIPKSSKPDRLKDINNWRPITIGSILLRLFSRIVTARLSKACPLNPRQRGFIRAAGCSENLKLLQTIIQSAKREHRPLGVVFVDIAKAFDTVSHQHIIHVLQQREVDPHIVGLVSNMYENISTYITTKRNTHTDKIQIRVGVKQGDPMSPLLFNLAMDPLLCKLEESGKGYHRGQSSITAMAFADDLVLLSDSWENMNTNISILETFCNLTGLKTQGQKCHGFYIKPTKDSYTINDCAAWTINGTPLNMIDPGESEKYLGLRFDPWIGIARSGLSTKLDFWLQRIDQAPLKPLQKTDILKTYTIPRLIYIADHSEVKTALLETLDQKIRTAVKEWLHLPPCTCDAILYSSTRDGGLGITKLAGLIPSVQARRLHRIAQSSDDTMKCFMEKEKMEQLHKKLWIQARGDRENIPSIWEAPPSSEPPNNVSTNSEWEAPTQKDKFPKPCNWRKNEFKKWTKLASQGRGIVNFERDKISNHWIQYYRRIPHRKLLTALQLRANVYPTREFLARGRQDQYIKACRHCDADIESCAHIIGNCPVTQDARIKRHNYICELLLEEAKKKDWVVFKEPHIRDSNKELYKPDLIFVKDARALVVDVTVRYEAAKSSLEEAAAEKVRKYKHLETEVRHLTNAKDVTFVGFPLGARGKWHQDNFKLLTELGLSKSRQVKMAETFSTVALFSSVDIVHMFASRARKSMVM

SEQ ID NO: 75 - protein, 1651 aa, synthetic construct
VTVKFKYKGEELEVDISKIKKVWRVGKMISFTYDDNGKTGRGAVSEKDAPKELLQMLEKSGKKASCPKPGPPVSAGAMSLESGLTTHSVLAIERGPNSLANSGSDFGGGGLGLPLRLLRVSVGTQTSRSDWVDLVSWSHPGPTSKSQQVDLVSLFPKHRVDLLSKNDQVDLVAQFLPSKFPPNLAENDLALLVNLEFYRSDLHVYECVHFAAHWEGLSGLPEVYEQLAPQPCVGETLHSSLPRDSELFVPEEGSSEKESEDAPKTSPPTPGKHGLEQTGEEKVMVTVPDKNPPCPCCGTRVNSVLNLIEHLKVSHGKRGVCFRCAKCGKENSNYHSVVCHFPKCRGPETEKAPAGEWICEVCNRDFTTKIGLGQHKRLAHPAVRNQERIVASQPKETSNRGARKRCWTKEEEELLIRLEAQFEGNKNINKLIAEHITTKTAKQISDKRRLLSRKPAEEPREEPGTCHHTRRAAASLRTEPEMSHHAQAEDRDNGGGDILAEAHGTRPDLTDQPLPDADHTWYTDGSSLLQEGQRKAGAAVTTETEVIWAKALPAGTSAQRAELIALTQALKMAEGKKLNVYTDSRYAFATAHIHGEIYRRRGWLTSEGKEIKNKDEILALLKALFLPKRLSIIHCPGHQKGHSAEARGNRMADQAARKAAITETPDTSTLLIENSSPSGGSKRTADGSEFEGGPGRRPLPGRAAAGGRTMDEIRRHPDKGNGQQRPTKQKSEEQLQAYYKKTLEERLSAGALNTFPRAFKQVMEGRDIKLVINQTAQDCFGCLESISQIRTATRDKKDTVTREKHPKKPFQKWMKDRAIKKGNYLRFQRLFYLDRGKLAKIILDDIECLSCDIPLSEIYSVFKTRWETTGSFKSLGDFKTYGKADNTAFRELITAKEIEKNVQEMSKGSAPGPDGITLGDVVKMDPEFSRTMEIFNLWLTTGKIPDMVRGCRTVLIPKSSKPDRLKDINNWRPITIGSILLRLFSRIVTARLSKACPLNPRQRGFIRAAGCSENLKLLQTIIQSAKREHRPLGVVFVDIAKAFDTVSHQHIIHVLQQREVDPHIVGLVSNMYENISTYITTKRNTHTDKIQIRVGVKQGDPMSPLLFNLAMDPLLCKLEESGKGYHRGQSSITAMAFADDLVLLSDSWENMNTNISILETFCNLTGLKTQGQKCHGFYIKPTKDSYTINDCAAWTINGTPLNMIDPGESEKYLGLRFDPWIGIARSGLSTKLDFWLQRIDQAPLKPLQKTDILKTYTIPRLIYIADHSEVKTALLETLDQKIRTAVKEWLHLPPCTCDAILYSSTRDGGLGITKLAGLIPSVQARRLHRIAQSSDDTMKCFMEKEKMEQLHKKLWIQARGDRENIPSIWEAPPSSEPPNNVSTNSEWEAPTQKDKFPKPCNWRKNEFKKWTKLASQGRGIVNFERDKISNHWIQYYRRIPHRKLLTALQLRANVYPTREFLARGRQDQYIKACRHCDADIESCAHIIGNCPVTQDARIKRHNYICELLLEEAKKKDWVVFKEPHIRDSNKELYKPDLIFVKDARALVVDVTVRYEAAKSSLEEAAAEKVRKYKHLETEVRHLTNAKDVTFVGFPLGARGKWHQDNFKLLTELGLSKSRQVKMAETFSTVALFSSVDIVHMFASRARKSMVM

SEQ ID NO: 76 - protein, 1651 aa, synthetic construct
VTVKFKYKGEELEVDISKIKKVWRVGKMISFTYDDNGKTGRGAVSEKDAPKELLQMLEKSGKKASCPKPGPPVSAGAMSLESGLTTHSVLAIERGPNSLANSGSDFGGGGLGLPLRLLRVSVGTQTSRSDWVDLVSWSHPGPTSKSQQVDLVSLFPKHRVDLLSKNDQVDLVAQFLPSKFPPNLAENDLALLVNLEFYRSDLHVYECVHFAAHWEGLSGLPEVYEQLAPQPCVGETLHSSLPRDSELFVPEEGSSEKESEDAPKTSPPTPGKHGLEQTGEEKVMVTVPDKNPPCPCCGTRVNSVLNLIEHLKVSHGKRGVCFRCAKCGKENSNYHSVVCHFPKCRGPETEKAPAGEWICEVCNRDFTTKIGLGQHKRLAHPAVRNQERIVASQPKETSNRGARKRCWTKEEEELLIRLEAQFEGNKNINKLIAEHITTKTAKQISDKRRLLSRKPAEEPREEPGTCHHTRRAAASLRTEPEMSHHAQAEDRDNGGGDILAEAHGTRPDLTDQPLPDADHTWYTDGSSLLQEGQRKAGAAVTTETEVIWAKALPAGTSAQRAELIALTQALKMAEGKKLNVYTDSRYAFATAHIHGEIYRRRGWLTSEGKEIKNKDEILALLKALFLPKRLSIIHCPGHQKGHSAEARGNRMADQAARKAAITETPDTSTLLIENSSPSGGSKRTADGSEFEGGPGRRPLPGRAAAGGRTMDEIRRHPDKGNGQQRPTKQKSEEQLQAYYKKTLEERLSAGALNTFPRAFKQVMEGRDIKLVINQTAQDCFGCLESISQIRTATRDKKDTVTREKHPKKPFQKWMKDRAIKKGNYLRFQRLFYLDRGKLAKIILDDIECLSCDIPLSEIYSVFKTRWETTGSFKSLGDFKTYGKADNTAFRELITAKEIEKNVQEMSKGSAPGPDGITLGDVVKMDPEFSRTMEIFNLWLTTGKIPDMVRGCRTVLIPKSSKPDRLKDINNWRPITIGSILLRLFSRIVTARLSKACPLNPRQRGFIRAAGCSENLKLLQTIIWSAKREHRPLGVVFVDIAKAFDTVSHQHIIHVLQQREVDPHIVGLVSNMYENISTYITTKRNTHTDKIQIRVGVKQGDPMSPLLFNLAMDPLLCKLEESGKGYHRGQSSITAMAFADDLVLLSDSWENMNTNISILETFCNLTGLKTQGQKCHGFYIKPTKDSYTINDCAAWTINGTPLNMIDPGESEKYLGLRFDPWIGIARSGLSTKLDFWLQRIDQAPLKPLQKTDILKTYTIPRLIYIADHSEVKTALLETLDQKIRTAVKEWLHLPPCTCDAILYSSTRDGGLGITKLAGLIPSVQARRLHRIAQSSDDTMKCFMEKEKMEQLHKKLWIQARGDRENIPSIWEAPPSSEPPNNVSTNSEWEAPTQKDKFPKPCNWRKNEFKKWTKLASQGRGIVNFERDKISNHWIQYYRRIPHRKLLTALQLRANVYPTREFLARGRQDQYIKACRHCDADIESCAHIIGNCPVTQDARIKRHNYICELLLEEAKKKDWVVFKEPHIRDSNKELYKPDLIFVKDARALVVDVTVRYEAAKSSLEEAAAEKVRKYKHLETEVRHLTNAKDVTFVGFPLGARGKWHQDNFKLLTELGLSKSRQVKMAETFSTVALFSSVDIVHMFASRARKSMVM

SEQ ID NO: 77 - protein, 1593 aa, synthetic construct
MPKRKVSSAEGAAKEEPKRRSARLSAKPPAKVEAKPKKAAAKDKSSDKKVQTKGKRGAKGKQAEVANQETKEDLPAENGETKTEESPASDEAGEKEAKSDASCPKPGPPVSAGAMSLESGLTTHSVLAIERGPNSLANSGSDFGGGGLGLPLRLLRVSVGTQTSRSDWVDLVSWSHPGPTSKSQQVDLVSLFPKHRVDLLSKNDQVDLVAQFLPSKFPPNLAENDLALLVNLEFYRSDLHVYECVHFAAHWEGLSGLPEVYEQLAPQPCVGETLHSSLPRDSELFVPEEGSSEKESEDAPKTSPPTPGKHGLEQTGEEKVMVTVPDKNPPCPCCGTRVNSVLNLIEHLKVSHGKRGVCFRCAKCGKENSNYHSVVCHFPKCRGPETEKAPAGEWICEVCNRDFTTKIGLGQHKRLAHPAVRNQERIVASQPKETSNRGAHKRCWTKEEEELLIRLEAQFEGNKNINKLIAEHITTKTAKQISDKRRLLSRKPAEEPREEPGTCHHTRRAAASLRTEPEMSHHAQAEDRDNGGGMPKRKVSSAEGAAKEEPKRRSARLSAKPPAKVEAKPKKAAAKDKSSDKKVQTKGKRGAKGKQAEVANQETKEDLPAENGETKTEESPASDEAGEKEAKSDGGPGRRPLPGRAAAGGRTMDEIRRHPDKGNGQQRPTKQKSEEQLQAYYKKTLEERLSAGALNTFPRAFKQVMEGRDIKLVINQTAQDCFGCLESISQIRTATRDKKDTVTREKHPKKPFQKWMKDRAIKKGNYLRFQRLFYLDRGKLAKIILDDIECLSCDIPLSEIYSVFKTRWETTGSFKSLGDFKTYGKADNTAFRELITAKEIEKNVQEMSKGSAPGPDGITLGDVVKMDPEFSRTMEIFNLWLTTGKIPDMVRGCRTVLIPKSSKPDRLKDINNWRPITIGSILLRLFSRIVTARLSKACPLNPRQRGFIRAAGCSENLKLLQTIIWSAKREHRPLGVVFVDIAKAFDTVSHQHIIHVLQQREVDPHIVGLVSNMYENISTYITTKRNTHTDKIQIRVGVKQGDPMSPLLFNLAMDPLLCKLEESGKGYHRGQSSITAMAFADDLVLLSDSWENMNTNISILETFCNLTGLKTQGQKCHGFYIKPTKDSYTINDCAAWTINGTPLNMIDPGESEKYLGLRFDPWIGIARSGLSTKLDFWLQRIDQAPLKPLQKTDILKTYTIPRLIYIADHSEVKTALLETLDQKIRTAVKEWLHLPPCTCDAILYSSTRDGGLGITKLAGLIPSVQARRLHRIAQSSDDTMKCFMEKEKMEQLHKKLWIQARGDRENIPSIWEAPPSSEPPNNVSTNSEWEAPTQKDKFPKPCNWRKNEFKKWTKLASQGRGIVNFERDKISNHWIQYYRRIPHRKLLTALQLRANVYPTREFLARGRQDQYIKACRHCDADIESCAHIIGNCPVTQDARIKRHNYICELLLEEAKKKDWVVFKEPHIRDSNKELYKPDLIFVKDARALVVDVTVRYEAAKSSLEEAAAEKVRKYKHLETEVRHLTNAKDVTFVGFPLGARGKWHQDNFKLLTELGLSKSRQVKMAETFSTVALFSSVDIVHMFASRARKSMVM

SEQ ID NO: 78 - protein, 1593 aa, synthetic construct
MPKRKVSSAEGAAKEEPKRRSARLSAKPPAKVEAKPKKAAAKDKSSDKKVQTKGKRGAKGKQAEVANQETKEDLPAENGETKTEESPASDEAGEKEAKSDASCPKPGPPVSAGAMSLESGLTTHSVLAIERGPNSLANSGSDFGGGGLGLPLRLLRVSVGTQTSRSDWVDLVSWSHPGPTSKSQQVDLVSLFPKHRVDLLSKNDQVDLVAQFLPSKFPPNLAENDLALLVNLEFYRSDLHVYECVHFAAHWEGLSGLPEVYEQLAPQPCVGETLHSSLPRDSELFVPEEGSSEKESEDAPKTSPPTPGKHGLEQTGEEKVMVTVPDKNPPCPCCGTRVNSVLNLIEHLKVSHGKRGVCFRCAKCGKENSNYHSVVCHFPKCRGPETEKAPAGEWICEVCNRDFTTKIGLGQHKRLAHPAVRNQERIVASQPKETSNRGAHKRCWTKEEEELLIRLEAQFEGNKNINKLIAEHITTKTAKQISDKRRLLSRKPAEEPREEPGTCHHTRRAAASLRTEPEMSHHAQAEDRDNGGGMPKRKVSSAEGAAKEEPKRRSARLSAKPPAKVEAKPKKAAAKDKSSDKKVQTKGKRGAKGKQAEVANQETKEDLPAENGETKTEESPASDEAGEKEAKSDGGPGRRPLPGRAAAGGRTMDEIRRHPDKGNGQQRPTKQKSEEQLQAYYKKTLEERLSAGALNTFPRAFKQVMEGRDIKLVINQTAQDCFGCLESISQIRTATRDKKDTVTREKHPKKPFQKWMKDRAIKKGNYLRFQRLFYLDRGKLAKIILDDIECLSCDIPLSEIYSVFKTRWETTGSFKSLGDFKTYGKADNTAFRELITAKEIEKNVQEMSKGSAPGPDGITLGDVVKMDPEFSRTMEIFNLWLTTGKIPDMVRGCRTVLIPKSSKPDRLKDINNWRPITIGSILLRLFSRIVTARLSKACPLNPRQRGFIRAAGCSENLKLLQTIIQSAKREHRPLGVVFVDIAKAFDTVSHQHIIHVLQQREVDPHIVGLVSNMYENISTYITTKRNTHTDKIQIRVGVKQGDPMSPLLFNLAMDPLLCKLEESGKGYHRGQSSITAMAFADDLVLLSDSWENMNTNISILETFCNLTGLKTQGQKCHGFYIKPTKDSYTINDCAAWTINGTPLNMIDPGESEKYLGLRFDPWIGIARSGLSTKLDFWLQRIDQAPLKPLQKTDILKTYTIPRLIYIADHSEVKTALLETLDQKIRTAVKEWLHLPPCTCDAILYSSTRDGGLGITKLAGLIPSVQARRLHRIAQSSDDTMKCFMEKEKMEQLHKKLWIQARGDRENIPSIWEAPPSSEPPNNVSTNSEWEAPTQKDKFPKPCNWRKNEFKKWTKLASQGRGIVNFERDKISNHWIQYYRRIPHRKLLTALQLRANVYPTREFLARGRQDQYIKACRHCDADIESCAHIIGNCPVTQDARIKRHNYICELLLEEAKKKDWVVFKEPHIRDSNKELYKPDLIFVKDARALVVDVTVRYEAAKSSLEEAAAEKVRKYKHLETEVRHLTNAKDVTFVGFPLGARGKWHQDNFKLLTELGLSKSRQVKMAETFSTVALFSSVDIVHMFASRARKSMVM

SEQ ID NO: 79 - protein, 1593 aa, synthetic construct
MPKRKVSSAEGAAKEEPKRRSARLSAKPPAKVEAKPKKAAAKDKSSDKKVQTKGKRGAKGKQAEVANQETKEDLPAENGETKTEESPASDEAGEKEAKSDASCPKPGPPVSAGAMSLESGLTTHSVLAIERGPNSLANSGSDFGGGGLGLPLRLLRVSVGTQTSRSDWVDLVSWSHPGPTSKSQQVDLVSLFPKHRVDLLSKNDQVDLVAQFLPSKFPPNLAENDLALLVNLEFYRSDLHVYECVHFAAHWEGLSGLPEVYEQLAPQPCVGETLHSSLPRDSELFVPEEGSSEKESEDAPKTSPPTPGKHGLEQTGEEKVMVTVPDKNPPCPCCGTRVNSVLNLIEHLKVSHGKRGVCFRCAKCGKENSNYHSVVCHFPKCRGPETEKAPAGEWICEVCNRDFTTKIGLGQHKRLAHPAVRNQERIVASQPKETSNRGARKRCWTKEEEELLIRLEAQFEGNKNINKLIAEHITTKTAKQISDKRRLLSRKPAEEPREEPGTCHHTRRAAASLRTEPEMSHHAQAEDRDNGGGMPKRKVSSAEGAAKEEPKRRSARLSAKPPAKVEAKPKKAAAKDKSSDKKVQTKGKRGAKGKQAEVANQETKEDLPAENGETKTEESPASDEAGEKEAKSDGGPGRRPLPGRAAAGGRTMDEIRRHPDKGNGQQRPTKQKSEEQLQAYYKKTLEERLSAGALNTFPRAFKQVMEGRDIKLVINQTAQDCFGCLESISQIRTATRDKKDTVTREKHPKKPFQKWMKDRAIKKGNYLRFQRLFYLDRGKLAKIILDDIECLSCDIPLSEIYSVFKTRWETTGSFKSLGDFKTYGKADNTAFRELITAKEIEKNVQEMSKGSAPGPDGITLGDVVKMDPEFSRTMEIFNLWLTTGKIPDMVRGCRTVLIPKSSKPDRLKDINNWRPITIGSILLRLFSRIVTARLSKACPLNPRQRGFIRAAGCSENLKLLQTIIQSAKREHRPLGVVFVDIAKAFDTVSHQHIIHVLQQREVDPHIVGLVSNMYENISTYITTKRNTHTDKIQIRVGVKQGDPMSPLLFNLAMDPLLCKLEESGKGYHRGQSSITAMAFADDLVLLSDSWENMNTNISILETFCNLTGLKTQGQKCHGFYIKPTKDSYTINDCAAWTINGTPLNMIDPGESEKYLGLRFDPWIGIARSGLSTKLDFWLQRIDQAPLKPLQKTDILKTYTIPRLIYIADHSEVKTALLETLDQKIRTAVKEWLHLPPCTCDAILYSSTRDGGLGITKLAGLIPSVQARRLHRIAQSSDDTMKCFMEKEKMEQLHKKLWIQARGDRENIPSIWEAPPSSEPPNNVSTNSEWEAPTQKDKFPKPCNWRKNEFKKWTKLASQGRGIVNFERDKISNHWIQYYRRIPHRKLLTALQLRANVYPTREFLARGRQDQYIKACRHCDADIESCAHIIGNCPVTQDARIKRHNYICELLLEEAKKKDWVVFKEPHIRDSNKELYKPDLIFVKDARALVVDVTVRYEAAKSSLEEAAAEKVRKYKHLETEVRHLTNAKDVTFVGFPLGARGKWHQDNFKLLTELGLSKSRQVKMAETFSTVALFSSVDIVHMFASRARKSMVM

SEQ ID NO: 80 - protein, 1593 aa, synthetic construct
MPKRKVSSAEGAAKEEPKRRSARLSAKPPAKVEAKPKKAAAKDKSSDKKVQTKGKRGAKGKQAEVANQETKEDLPAENGETKTEESPASDEAGEKEAKSDASCPKPGPPVSAGAMSLESGLTTHSVLAIERGPNSLANSGSDFGGGGLGLPLRLLRVSVGTQTSRSDWVDLVSWSHPGPTSKSQQVDLVSLFPKHRVDLLSKNDQVDLVAQFLPSKFPPNLAENDLALLVNLEFYRSDLHVYECVHFAAHWEGLSGLPEVYEQLAPQPCVGETLHSSLPRDSELFVPEEGSSEKESEDAPKTSPPTPGKHGLEQTGEEKVMVTVPDKNPPCPCCGTRVNSVLNLIEHLKVSHGKRGVCFRCAKCGKENSNYHSVVCHFPKCRGPETEKAPAGEWICEVCNRDFTTKIGLGQHKRLAHPAVRNQERIVASQPKETSNRGARKRCWTKEEEELLIRLEAQFEGNKNINKLIAEHITTKTAKQISDKRRLLSRKPAEEPREEPGTCHHTRRAAASLRTEPEMSHHAQAEDRDNGGGMPKRKVSSAEGAAKEEPKRRSARLSAKPPAKVEAKPKKAAAKDKSSDKKVQTKGKRGAKGKQAEVANQETKEDLPAENGETKTEESPASDEAGEKEAKSDGGPGRRPLPGRAAAGGRTMDEIRRHPDKGNGQQRPTKQKSEEQLQAYYKKTLEERLSAGALNTFPRAFKQVMEGRDIKLVINQTAQDCFGCLESISQIRTATRDKKDTVTREKHPKKPFQKWMKDRAIKKGNYLRFQRLFYLDRGKLAKIILDDIECLSCDIPLSEIYSVFKTRWETTGSFKSLGDFKTYGKADNTAFRELITAKEIEKNVQEMSKGSAPGPDGITLGDVVKMDPEFSRTMEIFNLWLTTGKIPDMVRGCRTVLIPKSSKPDRLKDINNWRPITIGSILLRLFSRIVTARLSKACPLNPRQRGFIRAAGCSENLKLLQTIIWSAKREHRPLGVVFVDIAKAFDTVSHQHIIHVLQQREVDPHIVGLVSNMYENISTYITTKRNTHTDKIQIRVGVKQGDPMSPLLFNLAMDPLLCKLEESGKGYHRGQSSITAMAFADDLVLLSDSWENMNTNISILETFCNLTGLKTQGQKCHGFYIKPTKDSYTINDCAAWTINGTPLNMIDPGESEKYLGLRFDPWIGIARSGLSTKLDFWLQRIDQAPLKPLQKTDILKTYTIPRLIYIADHSEVKTALLETLDQKIRTAVKEWLHLPPCTCDAILYSSTRDGGLGITKLAGLIPSVQARRLHRIAQSSDDTMKCFMEKEKMEQLHKKLWIQARGDRENIPSIWEAPPSSEPPNNVSTNSEWEAPTQKDKFPKPCNWRKNEFKKWTKLASQGRGIVNFERDKISNHWIQYYRRIPHRKLLTALQLRANVYPTREFLARGRQDQYIKACRHCDADIESCAHIIGNCPVTQDARIKRHNYICELLLEEAKKKDWVVFKEPHIRDSNKELYKPDLIFVKDARALVVDVTVRYEAAKSSLEEAAAEKVRKYKHLETEVRHLTNAKDVTFVGFPLGARGKWHQDNFKLLTELGLSKSRQVKMAETFSTVALFSSVDIVHMFASRARKSMVM

SEQ ID NO: 81 - protein, 1697 aa, synthetic construct
MPKRKVSSAEGAAKEEPKRRSARLSAKPPAKVEAKPKKAAAKDKSSDKKVQTKGKRGAKGKQAEVANQETKEDLPAENGETKTEESPASDEAGEKEAKSDASCPKPGPPVSAGAMSLESGLTTHSVLAIERGPNSLANSGSDFGGGGLGLPLRLLRVSVGTQTSRSDWVDLVSWSHPGPTSKSQQVDLVSLFPKHRVDLLSKNDQVDLVAQFLPSKFPPNLAENDLALLVNLEFYRSDLHVYECVHFAAHWEGLSGLPEVYEQLAPQPCVGETLHSSLPRDSELFVPEEGSSEKESEDAPKTSPPTPGKHGLEQTGEEKVMVTVPDKNPPCPCCGTRVNSVLNLIEHLKVSHGKRGVCFRCAKCGKENSNYHSVVCHFPKCRGPETEKAPAGEWICEVCNRDFTTKIGLGQHKRLAHPAVRNQERIVASQPKETSNRGAHKRCWTKEEEELLIRLEAQFEGNKNINKLIAEHITTKTAKQISDKRRLLSRKPAEEPREEPGTCHHTRRAAASLRTEPEMSHHAQAEDRDNGGGMPKRKVSSAEGAAKEEPKRRSARLSAKPPAKVEAKPKKAAAKDKSSDKKVQTKGKRGAKGKQAEVANQETKEDLPAENGETKTEESPASDEAGEKEAKSDGGPGRRPLPGRAAAGGRTMDEIRRHPDKGNGQQRPTKQKSEEQLQAYYKKTLEERLSAGALNTFPRAFKQVMEGRDIKLVINQTAQDCFGCLESISQIRTATRDKKDTVTREKHPKKPFQKWMKDRAIKKGNYLRFQRLFYLDRGKLAKIILDDIECLSCDIPLSEIYSVFKTRWETTGSFKSLGDFKTYGKADNTAFRELITAKEIEKNVQEMSKGSAPGPDGITLGDVVKMDPEFSRTMEIFNLWLTTGKIPDMVRGCRTVLIPKSSKPDRLKDINNWRPITIGSILLRLFSRIVTARLSKACPLNPRQRGFIRAAGCSENLKLLQTIIWSAKREHRPLGVVFVDIAKAFDTVSHQHIIHVLQQREVDPHIVGLVSNMYENISTYITTKRNTHTDKIQIRVGVKQGDPMSPLLFNLAMDPLLCKLEESGKGYHRGQSSITAMAFADDLVLLSDSWENMNTNISILETFCNLTGLKTQGQKCHGFYIKPTKDSYTINDCAAWTINGTPLNMIDPGESEKYLGLRFDPWIGIARSGLSTKLDFWLQRIDQAPLKPLQKTDILKTYTIPRLIYIADHSEVKTALLETLDQKIRTAVKEWLHLPPCTCDAILYSSTRDGGLGITKLAGLIPSVQARRLHRIAQSSDDTMKCFMEKEKMEQLHKKLWIQARGDRENIPSIWEAPPGGMPKRKVSSAEGAAKEEPKRRSARLSAKPPAKVEAKPKKAAAKDKSSDKKVQTKGKRGAKGKQAEVANQETKEDLPAENGETKTEESPASDEAGEKEAKSDGGSSEPPNNVSTNSEWEAPTQKDKFPKPCNWRKNEFKKWTKLASQGRGIVNFERDKISNHWIQYYRRIPHRKLLTALQLRANVYPTREFLARGRQDQYIKACRHCDADIESCAHIIGNCPVTQDARIKRHNYICELLLEEAKKKDWVVFKEPHIRDSNKELYKPDLIFVKDARALVVDVTVRYEAAKSSLEEAAAEKVRKYKHLETEVRHLTNAKDVTFVGFPLGARGKWHQDNFKLLTELGLSKSRQVKMAETFSTVALFSSVDIVHMFASRARKSMVM

SEQ ID NO: 82 - protein, 1697 aa, synthetic construct
MPKRKVSSAEGAAKEEPKRRSARLSAKPPAKVEAKPKKAAAKDKSSDKKVQTKGKRGAKGKQAEVANQETKEDLPAENGETKTEESPASDEAGEKEAKSDASCPKPGPPVSAGAMSLESGLTTHSVLAIERGPNSLANSGSDFGGGGLGLPLRLLRVSVGTQTSRSDWVDLVSWSHPGPTSKSQQVDLVSLFPKHRVDLLSKNDQVDLVAQFLPSKFPPNLAENDLALLVNLEFYRSDLHVYECVHFAAHWEGLSGLPEVYEQLAPQPCVGETLHSSLPRDSELFVPEEGSSEKESEDAPKTSPPTPGKHGLEQTGEEKVMVTVPDKNPPCPCCGTRVNSVLNLIEHLKVSHGKRGVCFRCAKCGKENSNYHSVVCHFPKCRGPETEKAPAGEWICEVCNRDFTTKIGLGQHKRLAHPAVRNQERIVASQPKETSNRGAHKRCWTKEEEELLIRLEAQFEGNKNINKLIAEHITTKTAKQISDKRRLLSRKPAEEPREEPGTCHHTRRAAASLRTEPEMSHHAQAEDRDNGGGMPKRKVSSAEGAAKEEPKRRSARLSAKPPAKVEAKPKKAAAKDKSSDKKVQTKGKRGAKGKQAEVANQETKEDLPAENGETKTEESPASDEAGEKEAKSDGGPGRRPLPGRAAAGGRTMDEIRRHPDKGNGQQRPTKQKSEEQLQAYYKKTLEERLSAGALNTFPRAFKQVMEGRDIKLVINQTAQDCFGCLESISQIRTATRDKKDTVTREKHPKKPFQKWMKDRAIKKGNYLRFQRLFYLDRGKLAKIILDDIECLSCDIPLSEIYSVFKTRWETTGSFKSLGDFKTYGKADNTAFRELITAKEIEKNVQEMSKGSAPGPDGITLGDVVKMDPEFSRTMEIFNLWLTTGKIPDMVRGCRTVLIPKSSKPDRLKDINNWRPITIGSILLRLFSRIVTARLSKACPLNPRQRGFIRAAGCSENLKLLQTIIQSAKREHRPLGVVFVDIAKAFDTVSHQHIIHVLQQREVDPHIVGLVSNMYENISTYITTKRNTHTDKIQIRVGVKQGDPMSPLLFNLAMDPLLCKLEESGKGYHRGQSSITAMAFADDLVLLSDSWENMNTNISILETFCNLTGLKTQGQKCHGFYIKPTKDSYTINDCAAWTINGTPLNMIDPGESEKYLGLRFDPWIGIARSGLSTKLDFWLQRIDQAPLKPLQKTDILKTYTIPRLIYIADHSEVKTALLETLDQKIRTAVKEWLHLPPCTCDAILYSSTRDGGLGITKLAGLIPSVQARRLHRIAQSSDDTMKCFMEKEKMEQLHKKLWIQARGDRENIPSIWEAPPGGMPKRKVSSAEGAAKEEPKRRSARLSAKPPAKVEAKPKKAAAKDKSSDKKVQTKGKRGAKGKQAEVANQETKEDLPAENGETKTEESPASDEAGEKEAKSDGGSSEPPNNVSTNSEWEAPTQKDKFPKPCNWRKNEFKKWTKLASQGRGIVNFERDKISNHWIQYYRRIPHRKLLTALQLRANVYPTREFLARGRQDQYIKACRHCDADIESCAHIIGNCPVTQDARIKRHNYICELLLEEAKKKDWVVFKEPHIRDSNKELYKPDLIFVKDARALVVDVTVRYEAAKSSLEEAAAEKVRKYKHLETEVRHLTNAKDVTFVGFPLGARGKWHQDNFKLLTELGLSKSRQVKMAETFSTVALFSSVDIVHMFASRARKSMVM

SEQ ID NO: 83 - protein, 1697 aa, synthetic construct
MPKRKVSSAEGAAKEEPKRRSARLSAKPPAKVEAKPKKAAAKDKSSDKKVQTKGKRGAKGKQAEVANQETKEDLPAENGETKTEESPASDEAGEKEAKSDASCPKPGPPVSAGAMSLESGLTTHSVLAIERGPNSLANSGSDFGGGGLGLPLRLLRVSVGTQTSRSDWVDLVSWSHPGPTSKSQQVDLVSLFPKHRVDLLSKNDQVDLVAQFLPSKFPPNLAENDLALLVNLEFYRSDLHVYECVHFAAHWEGLSGLPEVYEQLAPQPCVGETLHSSLPRDSELFVPEEGSSEKESEDAPKTSPPTPGKHGLEQTGEEKVMVTVPDKNPPCPCCGTRVNSVLNLIEHLKVSHGKRGVCFRCAKCGKENSNYHSVVCHFPKCRGPETEKAPAGEWICEVCNRDFTTKIGLGQHKRLAHPAVRNQERIVASQPKETSNRGARKRCWTKEEEELLIRLEAQFEGNKNINKLIAEHITTKTAKQISDKRRLLSRKPAEEPREEPGTCHHTRRAAASLRTEPEMSHHAQAEDRDNGGGMPKRKVSSAEGAAKEEPKRRSARLSAKPPAKVEAKPKKAAAKDKSSDKKVQTKGKRGAKGKQAEVANQETKEDLPAENGETKTEESPASDEAGEKEAKSDGGPGRRPLPGRAAAGGRTMDEIRRHPDKGNGQQRPTKQKSEEQLQAYYKKTLEERLSAGALNTFPRAFKQVMEGRDIKLVINQTAQDCFGCLESISQIRTATRDKKDTVTREKHPKKPFQKWMKDRAIKKGNYLRFQRLFYLDRGKLAKIILDDIECLSCDIPLSEIYSVFKTRWETTGSFKSLGDFKTYGKADNTAFRELITAKEIEKNVQEMSKGSAPGPDGITLGDVVKMDPEFSRTMEIFNLWLTTGKIPDMVRGCRTVLIPKSSKPDRLKDINNWRPITIGSILLRLFSRIVTARLSKACPLNPRQRGFIRAAGCSENLKLLQTIIQSAKREHRPLGVVFVDIAKAFDTVSHQHIIHVLQQREVDPHIVGLVSNMYENISTYITTKRNTHTDKIQIRVGVKQGDPMSPLLFNLAMDPLLCKLEESGKGYHRGQSSITAMAFADDLVLLSDSWENMNTNISILETFCNLTGLKTQGQKCHGFYIKPTKDSYTINDCAAWTINGTPLNMIDPGESEKYLGLRFDPWIGIARSGLSTKLDFWLQRIDQAPLKPLQKTDILKTYTIPRLIYIADHSEVKTALLETLDQKIRTAVKEWLHLPPCTCDAILYSSTRDGGLGITKLAGLIPSVQARRLHRIAQSSDDTMKCFMEKEKMEQLHKKLWIQARGDRENIPSIWEAPPGGMPKRKVSSAEGAAKEEPKRRSARLSAKPPAKVEAKPKKAAAKDKSSDKKVQTKGKRGAKGKQAEVANQETKEDLPAENGETKTEESPASDEAGEKEAKSDGGSSEPPNNVSTNSEWEAPTQKDKFPKPCNWRKNEFKKWTKLASQGRGIVNFERDKISNHWIQYYRRIPHRKLLTALQLRANVYPTREFLARGRQDQYIKACRHCDADIESCAHIIGNCPVTQDARIKRHNYICELLLEEAKKKDWVVFKEPHIRDSNKELYKPDLIFVKDARALVVDVTVRYEAAKSSLEEAAAEKVRKYKHLETEVRHLTNAKDVTFVGFPLGARGKWHQDNFKLLTELGLSKSRQVKMAETFSTVALFSSVDIVHMFASRARKSMVM

SEQ ID NO: 84 - protein, 1697 aa, synthetic construct
MPKRKVSSAEGAAKEEPKRRSARLSAKPPAKVEAKPKKAAAKDKSSDKKVQTKGKRGAKGKQAEVANQETKEDLPAENGETKTEESPASDEAGEKEAKSDASCPKPGPPVSAGAMSLESGLTTHSVLAIERGPNSLANSGSDFGGGGLGLPLRLLRVSVGTQTSRSDWVDLVSWSHPGPTSKSQQVDLVSLFPKHRVDLLSKNDQVDLVAQFLPSKFPPNLAENDLALLVNLEFYRSDLHVYECVHFAAHWEGLSGLPEVYEQLAPQPCVGETLHSSLPRDSELFVPEEGSSEKESEDAPKTSPPTPGKHGLEQTGEEKVMVTVPDKNPPCPCCGTRVNSVLNLIEHLKVSHGKRGVCFRCAKCGKENSNYHSVVCHFPKCRGPETEKAPAGEWICEVCNRDFTTKIGLGQHKRLAHPAVRNQERIVASQPKETSNRGARKRCWTKEEEELLIRLEAQFEGNKNINKLIAEHITTKTAKQISDKRRLLSRKPAEEPREEPGTCHHTRRAAASLRTEPEMSHHAQAEDRDNGGGMPKRKVSSAEGAAKEEPKRRSARLSAKPPAKVEAKPKKAAAKDKSSDKKVQTKGKRGAKGKQAEVANQETKEDLPAENGETKTEESPASDEAGEKEAKSDGGPGRRPLPGRAAAGGRTMDEIRRHPDKGNGQQRPTKQKSEEQLQAYYKKTLEERLSAGALNTFPRAFKQVMEGRDIKLVINQTAQDCFGCLESISQIRTATRDKKDTVTREKHPKKPFQKWMKDRAIKKGNYLRFQRLFYLDRGKLAKIILDDIECLSCDIPLSEIYSVFKTRWETTGSFKSLGDFKTYGKADNTAFRELITAKEIEKNVQEMSKGSAPGPDGITLGDVVKMDPEFSRTMEIFNLWLTTGKIPDMVRGCRTVLIPKSSKPDRLKDINNWRPITIGSILLRLFSRIVTARLSKACPLNPRQRGFIRAAGCSENLKLLQTIIWSAKREHRPLGVVFVDIAKAFDTVSHQHIIHVLQQREVDPHIVGLVSNMYENISTYITTKRNTHTDKIQIRVGVKQGDPMSPLLFNLAMDPLLCKLEESGKGYHRGQSSITAMAFADDLVLLSDSWENMNTNISILETFCNLTGLKTQGQKCHGFYIKPTKDSYTINDCAAWTINGTPLNMIDPGESEKYLGLRFDPWIGIARSGLSTKLDFWLQRIDQAPLKPLQKTDILKTYTIPRLIYIADHSEVKTALLETLDQKIRTAVKEWLHLPPCTCDAILYSSTRDGGLGITKLAGLIPSVQARRLHRIAQSSDDTMKCFMEKEKMEQLHKKLWIQARGDRENIPSIWEAPPGGMPKRKVSSAEGAAKEEPKRRSARLSAKPPAKVEAKPKKAAAKDKSSDKKVQTKGKRGAKGKQAEVANQETKEDLPAENGETKTEESPASDEAGEKEAKSDGGSSEPPNNVSTNSEWEAPTQKDKFPKPCNWRKNEFKKWTKLASQGRGIVNFERDKISNHWIQYYRRIPHRKLLTALQLRANVYPTREFLARGRQDQYIKACRHCDADIESCAHIIGNCPVTQDARIKRHNYICELLLEEAKKKDWVVFKEPHIRDSNKELYKPDLIFVKDARALVVDVTVRYEAAKSSLEEAAAEKVRKYKHLETEVRHLTNAKDVTFVGFPLGARGKWHQDNFKLLTELGLSKSRQVKMAETFSTVALFSSVDIVHMFASRARKSMVM

SEQ ID NO: 85 - protein, 118 aa, synthetic construct
MASGRDPREPLPGWLEIWDLDREPWDEWLQDMLRDLNEEARRHFGMNMLIRVWNYCVEEGRRHNTPWNEIGYKYYRIVQKSMFVHFRCGCRRRGPFSPYEERRNGQGGGAPPPPPGLA

SEQ ID NO: 86 - protein, 99 aa, synthetic construct
MAEGAPEIPEGAGEVDLNTWLERSLEKINQEARLHFHPEFLFRLWNACIEHWHDRHQRSLSYAKYRYLLLMNKAMFTHMQQECPCRSGHPRGPPPPGMV

SEQ ID NO: 87 - protein, 113 aa, synthetic construct
MTDPRERVPPGNSGEETIGEAFEWLERTIEALNREAVNHLPRELIFQVWQRSWRYWHDEQGMSASYTKYRYLCLMQKAIFTHFKRGCTCWGEDMGREGLEDQGPPPPPPPGLV

SEQ ID NO: 88 - protein, 136 aa, synthetic construct
KRSPDKQMAVLPRRERNRQAAAANPENSRGKGRRGQRGKNRGCVLTAIHLNVTDLGLGYETKEELIFRYCSGSCDAAETTYDKILKNLSRNRRLVSDKVGQACCRPIAFDDDLSFLDDNLVYHILRKHSAKRCGCI

SEQ ID NO: 89 - protein, 193 aa, synthetic construct
MGVHECPAWLWLLLSLLSLPLGLPVLGAPPRLICDSRVLERYLLEAKEAENITTGCAEHCSLNENITVPDTKVNFYAWKRMEVGQQAVEVWQGLALLSEAVLRGQALLVNSSQPWEPLQLHVDKAVSGLRSLTTLLRALGAQKEAISPPDAASAAPLRTITADTFRKLFRVYSNFLRGKLKLYTGEACRTGDR